European Patent Specification EP 3 234 136 B1, published August 21, 2024. Title: METHODS AND COMPOSITIONS FOR IN VITRO VIRAL GENOME ENGINEERING. Applicant: SYNTHETIC GENOMICS, INC. DIPETRILLO, Christen CADY, Kyle C. BARBU, Elana M. The sequence listing filed with the application follows.

SEQUENCE LISTING (51 sequences)

SEQ ID NO: 1 - DNA, 288 bp, Phikmvlikevirus LUZ19
  misc_feature: Wild type LUZ19 gp13
gtgctggccctcggtgccttcgacctgtccggcctgatggtaggttcctgcctcgtagtaggtggtgagctgaaggccctgtgcgttgatgaccggcacagcaggcagggtatcggcgctgagctggtacgggccgctgagctggctggtgccgagtatctgacctgcttcgagttcctggagccgttctacgccgacttgggctggagcaccacccaccgcgaggcgaactggacagcaggagagccggacgtgctgcacatgagggcacccggtcatgacgtatga

SEQ ID NO: 2 - DNA, 756 bp, Phikmvlikevirus LUZ19
  misc_feature: Wild type LUZ19 gp38
gtggctcggttcaagaatcccgagaccatccacgttgcagatggggtcgaggctgtcttcagtctcgacttcccgttcctgcggcgtgaggacgtattcgtccaggtcgataagatactcgtcaccgactatacgtgggtagacgacaccaacatccaattggccgtggtgccgaagaaggaccaagaggtccgcatcttccgcgacacgcccgcccaggtcccggacacacagttcagccaggacatcccgttcctgcctcgatacatcgacgcgaacaacaagcagctcctgtacgctgtgcaggaaggcatcaacaccgcgaacctcgctctcgatggcgtactcgacgcgatccgtatcgccgaggaggctcgtcgcctggcgcaggaagcactcgacgccgccaatgaggcgcttcgccgtgccctgggcttcgctgagattcgcaccgtgaccgaggactcggacatcgatccgagctggcgcggttactggaaccgttgcatcaccgccgataaacctctgaccctgaccatgcagatggaagacccggatgcaccgtgggtcgagttcagcgaggttcacttcgagcaggccggtgtgcgtgacctaaacatcgtagccggtcctggcgttaccatcaaccgtttgcagaacaccaccatgcagctctacggcgagaatggcgtgtgtactctcaagcggctgggcgctaaccactggatcgtgttcggggccatggaggacgaataa

SEQ ID NO: 3 - DNA, 906 bp, Phikmvlikevirus LUZ19
  misc_feature: Wild type LUZ19 gp40
atgtttaagaccgaagtaaagggacgttacaccctgattcgccgcaaggcggacggcactccggtggagactctggagttcgacaacatcattacgaatgcgggcctggattggatcgccgctatggataccgacctcatgggcgaacccgtagcggtcagcacttctacagccgatcccaacccgagcgcacccgccatcccggaggttgtgcaacgcacgtccgcatctgcccctggtggaggtactacgtcgggcctggatggcgagtggctgttctggcggaggcgttggagattcccgcagggcaccctagctggtcaagtcctggccaccgtgggcctcatctgcaactcggatcgtcgcttcgagagtaacacgggtgagctgatcccgaaggataccccgctgtcgtacactcgcatcaaggacgccgccgggcagcctactactctggtggtggccgctgacgagattctggatgtccagtacgagttccgcagccggcccgtaggaacggctgaggccaagttcgtgatctccggcgtggaacgcaccttccggctgatcccaaagccttttgcgaaccgtgctaatctctccggggaacgctacatcttctacaacaccaacccctacatcaacggcaaggacgcctccggcggcaatgtccgagacggtcagtggcagaagaaatatcccaagtacgtgcgcggctcctacaaggcgcagatcacgctgctggcccaggtccagaacggcaatatggctggcggcatcaccggcaccgaggaactccagatttacaatggacgtaactatgtgctcgatatcaacccgcctgttgtgaagaacaatacccaggagttcaccgtgaccctggagtttacggtggcgagggcataa

SEQ ID NO: 4 - DNA, 2481 bp, Phikmvlikevirus LUZ19
  misc_feature: Wild type LUZ19 gp34
atgagctacaagcaatccgcgtatcccaatctgctgatgggtgtgagccagcaggtgcccttcgagcgcctgccgggccagctcagcgagcagatcaacatggtatccgatcccgtgtcaggacttcggcggcgcagcggtatcgagctgatggcccacctgctgcataccgaccagccctggccgaggccgttcctctaccacacgaacctcggtggccgcagcattgcgatgctggtggcgcagcaccgtggcgagctgtacctgttcgacgagcgggacggtcgcctgctgatgggtcagcccctggtgcatgactacctcaaggccaacgattacaggcagctacgggccgccacggtggccgatgacctgttcatcgccaacctgagtgtaaagcccgaggccgaccgcaccgacatcaagggcgtagaccccaacaaggccggctggctgtacatcaaggcaggccagtattcgaaggcattctccatgaccatcaaggtcaaggacaacgccaccggcaccacctacagccacacggccacctacgtgacgccggacaacgccagcacgaaccccaacctcgctgaggcgccattccaaacgagcgtaggctacatcgcgtggcagctctacggcaagttcttcggtgcgccggagtacactctgcccaactcgacgaagaagtacccgaaggtagacccggacgccaacgcggcaaccatagccggttacctcaaccaacggggcgtgcaggacgggtacatcgcgttccgtggcgacgccgatatccacgttgaagtgtccacggacatgggcaacaactacggcatagcctccggcggtatgagcctcaacgccacggcagacctgccggccttactgccgggcgcgggtgctcctggcgtgggtgtgcagttcatggacggcgctgtcatggccaccggctccaccaaggccccggtatacttcgagtgggattccgctaaccgccgctgggcagagcgggccgcctacggcaccgattgggtcctgaagaagatgccactggccctgcgctgggatgaggctaccgacacctacagcttgaacgagctggagtatgatcgacgtggctccggcgacgaggatacgaaccccacgttcaacttcgtcacccgaggcatcaccggcatgacgaccttccagggtcgcctcgtcctcctgtcgcaggagtacgtctgcatgtcggccagtaacaatccacaccgctggttcaagaagtcggcagccgcgctgaacgacgatgatcctatcgagatcgcagcccaggggagcctgactgaaccgtacgagcacgcggtcaccttcaacaaggacttgatcgtcttcgccaagaagtatcaggccgtggtccccggtggcggcattgtaactccccggacggcggttatcagcatcaccacgcagtacgacctcgataccagggcggcacctgccgtgactggccgcagtgtgtacttcgctgcggagcgtgccctgggtttcatgggcctgcatgagatggccccgtctccgtccacggacagccactacgtcgccgaagacgttaccagccacatcccgagctacatgccggggcctgctgagtacatccaggcggcggcctccagcggctacctggtgttcggcaccagcacggcggacgagatgatctgccaccagtacctctggcagggcaacgagaaagtgcagaacgcgtttcatcgctggacgttgcggcatcagatcatcggcgcctacttcactggtgacaacctgatggttctgattcagaagggccaggagatcgccctgggacggatgcacctgaacagcctgccagcccgtgagggtctgcaataccctaaatacgactactggcggcgtatcgaggcgaccgtcgatggtgagctggaactgaccaagcagcattgggacctgatcaaggatgcctctgccgtgtaccagctacagcctgtggccggcgcctacatggagcgtacccatctcggcgtgaagcgcgagacgaatacgaaggtgttcctcgacgtgcccgaggccgtggtcggggcggtgtatgtggtcggctgcgagttctggtcgaaggtggagttcactccgccggttctccgggaccacaatggcctgcccatgacctcgacccgtgcagtgcttcatcggtacaacgtaaacttcggctggaccggcgagttcctgtggcgcatcagcgacacggctcgacccaaccagccgtggtacgacacgacgcccctccggttgttcagccggcaactcaatgccggggagcctctggtggatagcgctgtggtgccgctgccggcacgggtcgatatggccacgtccaagttcgagctgagctgtcacagtccgtacgacatgaacgttcgggctgtcgagtacaacttcaagtccaaccaaacctacaggagggtgtga

SEQ ID NO: 5 - protein, 826 aa, Phikmvlikevirus LUZ19
  misc_feature: Wild type LUZ19 Gp34 protein
MSYKQSAYPNLLMGVSQQVPFERLPGQLSEQINMVSDPVSGLRRRSGIELMAHLLHTDQPWPRPFLYHTNLGGRSIAMLVAQHRGELYLFDERDGRLLMGQPLVHDYLKANDYRQLRAATVADDLFIANLSVKPEADRTDIKGVDPNKAGWLYIKAGQYSKAFSMTIKVKDNATGTTYSHTATYVTPDNASTNPNLAEAPFQTSVGYIAWQLYGKFFGAPEYTLPNSTKKYPKVDPDANAATIAGYLNQRGVQDGYIAFRGDADIHVEVSTDMGNNYGIASGGMSLNATADLPALLPGAGAPGVGVQFMDGAVMATGSTKAPVYFEWDSANRRWAERAAYGTDWVLKKMPLALRWDEATDTYSLNELEYDRRGSGDEDTNPTFNFVTRGITGMTTFQGRLVLLSQEYVCMSASNNPHRWFKKSAAALNDDDPIEIAAQGSLTEPYEHAVTFNKDLIVFAKKYQAVVPGGGIVTPRTAVISITTQYDLDTRAAPAVTGRSVYFAAERALGFMGLHEMAPSPSTDSHYVAEDVTSHIPSYMPGPAEYIQAAASSGYLVFGTSTADEMICHQYLWQGNEKVQNAFHRWTLRHQIIGAYFTGDNLMVLIQKGQEIALGRMHLNSLPAREGLQYPKYDYWRRIEATVDGELELTKQHWDLIKDASAVYQLQPVAGAYMERTHLGVKRETNTKVFLDVPEAVVGAVYVVGCEFWSKVEFTPPVLRDHNGLPMTSTRAVLHRYNVNFGWTGEFLWRISDTARPNQPWYDTTPLRLFSRQLNAGEPLVDSAVVPLPARVDMATSKFELSCHSPYDMNVRAVEYNFKSNQTYRRV

SEQ ID NO: 6 - DNA, 1497 bp, Pseudomonas aeruginosa
atgtccaatgacaacgaagtacctggttccatggttattgtcgcacaaggtccagacgatcaatacgcatacgaggttccccctatcgatagcgcggccgttgccgggaatatgtttggcgacttaattcaaagagaaatatatctacagaaaaacatttattatccagtccgatctatttttgaacaaggaacaaaagaaaagaaggagatcaacaagaaagtatctgatcaagtcgatggcttgctaaagcagatcactcaaggaaaaagggaggccacaaggcaagagcgagtcgatgtcatgtcggcagtcctgcacaagatggaatctgatcttgaaggatacaaaaagacctttaccaaaggcccattcattgactacgaaaagcagtcaagcctctccatctatgaggcctgggtcaagatctgggagaagaactcttgggaagaaagaaagaagtacccttttcagcagcttgttagagatgaactggagcgggcggttgcctactacaaacaagattcactctctgaagcggtaaaagtgctaagacaggagctcaacaagcaaaaagcgctaaaggaaaaagaggacctctctcaactggagcgggactacagaacccgaaaggcgaatctcgagatgaaagtacaatccgagcttgatcaagcgggaagtgctttgcctccattggtcagtccaacgccagagcaatggcttgaacgtgccacaagactggttacgcaagcaattgctgataaaaagcagctgcagaccacaaacaatactcttatcaagaattccccaacccctctagaaaagcagaaagccatctacaatggtgagctacttgtggatgagatagccagtctacaggcccgcttagttaagctgaacgccgaaacgacacgacgcaggacagaagcagaacgcaaggcggccgaggaacaagcgttgcaagatgctattaaatttactgccgacttttataaggaagtaactgagaaatttggcgcacgaacatcggagatggcgcgccaactggccgaaggcgccagggggaaaaatatcaggagttcggcggaagcaatcaagtcgtttgaaaagcacaaggatgcgttaaataaaaaacttagccttaaagataggcaagccattgccaaagcctttgattctctagacaagcagatgatggcgaagagccttgagaaatttagcaaaggctttggagttgtaggcaaagctattgacgccgccagcctgtaccaagagttcaagatatctacggaaaccggggactggaaaccattctttgtaaaaattgaaacactagctgctggtgcggccgccagttggcttgtgggtattgcatttgccacggcaacagccactcctataggcattctggggttcgcactggtaatggcagttaccggggcgatgattgacgaagaccttctagaaaaagcaaacaatcttgtaatatccatttaa

SEQ ID NO: 7 - DNA, 345 bp, Phikmvlikevirus LKD16
gagtaccaactgaacacgagcgcaccctgcgctgcctgctccaagacatccacgggccgctgaatctgctgttcccaggtatccgggtgaaggtggaggaggcgtgcctcggatacttgggctacagggagcggggctattgggagctgcgcctccaggtggactacgaccacccgaagcttgggcacctccgctacagtcaggccgtgccggagtacgtgctgatcaacgaccgcgacagcatcatcaagtacctgatggaagcagtccctcggcaggtactagagggcatgctcaataaggcccaggaattcgtaaccaagaactggtattccctatgacgac

SEQ ID NO: 8 - DNA, 204 bp, Phikmvlikevirus phi-KF77
  misc_feature: Phi KF77 gp7 sequence added
tacaaggtggtgacgcctagctcggcagagggcgccgttgtgctggcgaccaagcagacgcctgccctcgctcaggcagtcatcgtactgcacagcatgaaccccgcgcagtacgcggtgggcacggccatactaaacacagactggcggtgccgccgcctgggtgccggcgagtacatcaagctcgttcaaggggaggccgac

SEQ ID NO: 9 - DNA, 60 bp, lambdalike lambda
  misc_feature: E. coli phage
atggttcgtgcaaacaaacgcaacgaggctcgttctgaacaaatccagatggagttctga

SEQ ID NO: 10 - DNA, 17757 bp, Cytomegalovirus HCMV
  misc_feature: HCMV fragment pre-editing
acgacggccagtgaattgtaatacgactcactatagggcgaattcgagctcggtacccgattaccctgttatccctaccattccgggccgtgtgctgggtccccgaggggcgggggggtgtttttagcgggggggtgaaatttggagtcttggagccgcgtgtgctgtggaggacggtgacggtggtaagagtgtgctgcggtgcggttgggacggcggcggcgaataaaagcggcgtgcggcgcgcacggcgaaaagcagacgcgcgtctgtgttgtgtgtctttgaccgcggcggaacacacgcggaaaagcgagtcccaggggacacacgacgagcgagtcccagggggggacgacgacggccagggacgcggaaacgacgcggaaaagaggaagtccccagggggacgggcggaaaagaggaagcgcctaggggaccgcgggggcaggaacagacgaagtacgccgcaacccgcgtcgaggacacacgcagaagcggccgcccaggggagggggggggggggactcgcgggccccggggcacacttgttgttccctccggccgccgacacgcaccccgaagccgcgcacaccgccgacacacccctgacacacccgcgacacacccgccacacgcccgacacacgcccgcgacacacccgaccgacacaccctgacacaccccgccaacacacccagccgcacccgccccgccaacacacccccgacacacccgacacacgcccgcgacacacccggcacacacccacccacccagccgcgcccccgacacaccccgaacggcgccggtgcgggacagggctcacggaggtttgcgggccgtgagcacgcctccctttgtacacactaccggtgcgtggcgtcccacgctatttgttcgcgagaccggactaagggaggtttgcggtgcgtcagcgcggggcggcgtttgcggcgtgtttcgaccagcgctttgtgcgcgctgcctgtgcgtgtcgtcccatggtctttgtcagcggcacggcgctggggacggggtttcaccgcgctgagggatctttctgcgggtgtgagggacggagcttttttcgcacgctgggcaccgggctgggggacggggggtgtgcgggacggcggtggggccggggcgttgcgggtacggggattacgctgggaacggggactcgcggacccgggctgagggacgggggtggcgggggtgtttgcggcgaggacgggggccttttgcggcggggacggggactcaccctcgcctatttaacctccacccacttcaacacacacatgccgcacaatcatgccagccacagacacaaacagcacccacaccacgccgcttcacccagagtaccaacacacgttacccttacaccacagcaacacacaaccgcctatccaaacctcggacaaacacgccaacgaagaacaccgcacgcagatggagctcgacgccgcggattacgctgcttgcgcgcaggcccgccaacacctctacgctcaaacacaaccccaactacacgcataccccaacgccaaccctcaggaaagcgctcatttttccacagaaaatcaacatcaactcacgcatctacttcacaacattggcgaaggcgcagcgctcggctaccccgtcccccgcgcggaaatccgccgcggcggtggcgactgggccgacagcgcgagcgacttcgacgccgactgctggtgcatgtggggacgcttcggaaccatgggccgccaacctatcgtgaccttactgttggcgcgccaacgcgacggcctcgctgactggaacgtcgtacgctgccgcggcacaggctttcgcgcacacgattccgaggacggcgtctctgtctggcgtcagcacttggtttttttactcggaggccacggccgccgtgtacagttagaacgtccatccgcgggagaagcccaagctcgaggcctattgccacgcatccggatcacccccatctccacatctccacgcccaaaaccaccccagcccaccatatccaccgcatcgcacccacatgctacgactcgcccacatcacacgctctttcctatcccttctacaccctcagccacggttcacaatccccgaaactacgccgtccaacttcacgccgaaacgacccgcacatggcgctgggcacgacgcggtgaacgtggcgcgtggatgccggccgagacatttacatgtcccaaggataaacgtccctggtagacggggtagggggatctaccagcccagggatcgcgtatttcgccgccacgctgcttcaccgatatccaataaacccatcccctcgccacgacgtctccgcgtatctttgtagcctcaggaatccgtccccacgtccatccatcccgagcactccacacgctataacagaccacggacacggcaaatgcatgcaaacttctcatttattgtgtctactactctgtgttgctacagggagtgaagggggtgaaggcaaagaaaaaaaaaaggaacaaaataatagattagcagaaggaataatccgtgcgaccgagcttgtgcttcttttcttataaggaggcaaatatactagggaaaacttaagaataggaagaaaccgaggtttgggagaaaagctgagataaaatagcgcattttccatacagaggttgttgtttttgtggatcctaagaggtttcaagtgcgaatctcaaagttctcacgagaatattgtcttcaagaatcgacaactgtggtccaagatttttttttggtctttttaggttctgcgagggacatcacgatggatcgttgcgatgaagtcacgcgtacgcctctggtgtggcgcggtgtcgtgacaggagagtgtgttttcagtgcagagctgtcttgattcctatatccgagtatctgttttctcgtaaggacggtaatcttctttggtgtaagtacatctaaaagctgcaaactatattttaagggctgtctctaggtgtactttgatgctggagtttttcgctgtgttgatgtgaataaatctactactactattatatgcagaaagagtgattatgccgagacaagattgcattggctgaactgtttcaaaaacgcctacactctacttatccgtaaacctaaggtaatactatgtgtaagttgtttttttttctttttgtagtaaaatggtgatacgtgcaattaaaactgtattccatgtttccatcctttcatttcaactttaaaggcggctttgagagcgaagaagtgcgaggataaaaatggatgactccttcgtgtccagggagtcgactactgcaacgctgattgattaaaagatggtctccgatgatgatgttgttattgatcgaatcatggtgcagaacggcgacggagaggagcgtgtccgccgccgggaaggtggtctctttctcttttcttttttcaagaaatcttccatgtgtttatcgtagtgatcgaaatcgactgatctcgggttctttttgttggtttcttttcggttaatcatgtattgttttctttttttacagaaagatacttttttcatgagcaattcctcgcccggcgccggcatgccgaggtggggccactgcgatcagcggcatgccgacgccgacccggggatcttggattcaccgttttctctcttctctctctacatacagaccgggtggcaggagcggtaaggaatcatcgtcgtctttcattcttcgatgattatggtaatactaaatcttatctaggagcatatacatctaagattggagtactagtagtcgtttgtggtttctattttttttatatttatctatgacagtttttctgtttttcgttttgataataatataataaaaactcatggacgtgaaatctggcttggttgtggtgatttcattctcattattgttgttttctttccgtcttgcggatgaagatgttgcgatgcggttgttgttggtgttgctatacaccgagagagatgatctttttgttcttctggttcatttcctatgattgtttggctgctgaccgacgcgtcaggatgtgcagggcatgcggggaatcaggaccggacacgggataatttcatctacctatacggagatcgcggtcctcgccatgaggatcgcgacaggcgcgtcgagggggcaggaacacccttgcggattgacattcttggtggtgtttcgttgttgtcggtagttgttgttgacgatgaggataaataaaaatgaccttgtttttgttctgttttctcttgttgggaatcgtcgactttgaattcttcgagttatcggaaagctgaggtacccaaatgtctgtagcttttttctttttaccctcttgtttatcatctgcgattcgtggtaggtaggagagggaaatgataatccgagattaaggaaaggagaagataaaaaataaaaaaaaaataataaaacagaagccgaccggccgccgacccgttccccaggaccagcctacgaggaatggataacgcggtggcgacggcagcggtggtggcgctgggggtggcggcagtggtactgctgatggtagtcgggacggaggagaggcgatgcatacatacacgcgtgcatgctgcatgggtggatggtacggccgggagacgcggaagagaaactcacataaaaaggtgacaaaaagagcggttgaaaaaagaaaacgagattcgaccagacagaagagaaggaccggggcttggcgacccttccacgactgctgttgtcatctcggctcccccgtcttctcccggccacgggcggctaagtcaccgccgttctccccatccgtccgagcgccgaccgaccagccggccgattcgcccgccggggcttctggagaacgccggggcagcagcgatctggggaagccgctaaacccctgcgtttttatatggtagctctgccgagcgcgggctgacgcgttgagtaagcggaaagacgtgtgtgacgaaaaggggtcccatggtatttcacgtgacgatgaggagatgcggtttggagcacatacggtttagaaaaagggagttgtcgtgacaagggctgagggacctctgtctccatgtgtgtataaaaagcaaggcacgttcataatgtaaaaaagaacacgttgtaaacaagctattgctgtatcattcggctgactatgcttcattcggactgattttcttttcctaacggcgtaacttaaagtgattaacgtatgatatttgttccccagagttatactatagtcatcatcctaaaattcagatataaatgaacacatgtcgtatgggattattaagaaaccgaaactctccacagttcaccatcttcttcgtcattcaaccgatgacccactccgtacaacgaatcagtctgctgtgtcacactgcaaactactagcgacgtatgcaaacaacttgaaacacgggctgttgtattgacgaccgttgtaccattactagtcacattgcatagagaccatccaccgtcatcccatctttcccacccgatggaaaaccgtcttctatcatcaactatggtaagatttcgaccctgcgaggtattcagtttccccatatccataacctggattttatcattaaaccccaatattaaacacttttttagtacccccccacccaccaaaaaatgtgactggaccggttcctagcagctctgggagccatgttcaggttgaaccacagctacagcgaaaccgagtccagtgaccggtaaccacgtccagcccctgcgtatgtaccagtccaagcacgtccggtcattgttctacacaggaaatctaactaggtcaacgcaattttattccaccgttacgcagaatactaacaaacaaacacacaaatttaacgaattacacgtagtttattacatgaaaactgtaagaacaccaattcactaagcgatacaacatttagctgacttccaagtgccacacatcaccactgtattcatccatgttttcaccgaaccaacgagacagatcgaagaagccagaatctcccgactttaaattacataaatccaacgtattatgaccacagctcgacacacaaatagttgcgttactattcacagtagcattacctatacccgtaacgttgcacaaccactgatcaccattgttaccaaaaacggttttccacttagttgtcaacggatctttcccatgcgtaatggtcaaattactaccagtcgtcgcttttagctcattacgagtattatccgcatccacatatatcaacgtcatagctaggcacgctataagtaccccccccccacaatggaatgttgccaaaccggttctttcccgttatagccatagcgttcccaggcaaaagcaaacgccaaacctaatgcagtgaaaagcgcttgcagccagaaccagcttatgtaccagccacaatcacatccggttattgtttccacaggaaatcctaccaggcaaagccccgcttgttttgttcctgaccatcttgtttagcaattcgtaaactgtcagcctagcgacgtccgtttagatcaaaagtcacgtatatagcgacgctgtttccacccgtttccccgtcccgccgtttccgaacaacccacccgggttcagacaaccgaccaccaacagaaatatacacacagaccaccgggagttcagttaaagatttcatcaggtttattttggctgctgctagtcttttgcttcttagaaaaaaaatacccatatagagaaataatgatagtttgacaacacatatggcagggatttcttcttcatcaataagatatgcaattcccccagggagagactttcaacaattgaatttacaaaaacaaaattacatcaggagaaagagaggatacattaataaatatattatatctggtgtatatactgaatgctgctggttcataaggtaacgatgctactttttttaattccaagatggtttttctttgttagtcttttgttgacttgctggttcctaaaagttcgcaaaaacgattgtgtgaagattatgacgttggttgactagttcatgagattctgctgtacgtgtgatggttattcgctggttcgttctaagatgagtatcgtactgtgtctgcgatggtcgtctcttactggcattctctcggctgcctcttgttttcatgattgaaaaggaaaaaaggactccgagggcgcggtcatcttttacttttcggttttctcgttggcgggtcagaggtagtcagatcatgagactgtcgtggtcgatgaaactgtgtctgctcaagtgacgtccatttcttgtacggagaaaaaagtcatcgggataaataaggctatacaaggcgttgtcaagcgtgcggctctaaacaaattaagcgatacaaaattacagtgatacgaataataaattaccccctccccctgtggtccccccgaggcgagagccacccatcgtgtactctcgcaccacccacgaccacagggggagacgggacgaagagacgacgcagagcgccatctcctcctggaggccggcggcgttaactgctacagctgcggcggcgacgacagctgcgatttgtcggccgacatgccgatggtatgggcggcggcggcggtggccgcggcagcggggaggagaggagagagaagaggagcggggcgtccgaaggcgaggatggcatggtctcgccggagcgcccggcttttatggaacactcgcgtccggttgggtatcacccacaggaagatgaatcacaacttccaaaccatcttgagacccgagtaacggtttacaggtcgcacgccagtctcagctaaaaacagcggacagtcccacgctgtttctgttgtggctctctccagtttcctcatcgccgtcttggtctccgtcatcatcggaagaataccacccgctctcatgcggcagtcgatcagcctcgatgaacgagacgcggcgacgcctttctacggccgactggttgtggtggtgaaagaagagcaccagcaatcccaggaggagcaacaagccctcacatgtccaggaggtcggggagagggcctgtcggagatgaccgtgaggcatcacgtacggcagctgaggagaaacggagaagaaaggaaaattaccgtcaggggccggggttcttattagagaaacagcacgtaggtcaggatccagatgctaatggcaatcatgatgacgatgatcatgcaggccaagacgcggcgcaccaatgcagaatccaatagccgccgtgcctccggttggtggccggcggcatctagagacatgatttgggggggggaccggcggcgcaaaaagacagggagatggacagtgccacggtgttttgttatgattaggacatggggaccggaagccgagacagagtactacagggtgttgaagggtaacgtgagggagatcatgtcatgggcgggctgaagaccgtgcggggaggatcgacgtgtgcggtgcttgtggaacacggtgttttaatatgtatccgcgtgtaatgcacgcggtgtgctttttagcactcggcttgataagctacgtgaccgtctgcgctgaaaccatggtcgccaccaactgtctcgtgaaaacagaaaatacccacctagcatgtaagtgcaatccgaatagtacatctaccaatggcagcaagtgccacgcgatgtgcaaatgccgggtcacagaacccattaccatgctaggcgcatactcggcctggggcgcgggctcgttcgtggccacgctgatagtcctgctggtggtcttcttcgtaatttacgcgcgcgaggaggagaaaaacaacacgggcaccgaggtagatcaatgtctggcctatcggagcctgacacgcaaaaagctggaacaacacgcggctaaaaagcagaacatctacgaacggattccataccgaccctccagacagaaagataactccccgttgatcgaaccgacgggcacagacgacgaagaggacgaggacgacgacgtttaacgaggaagacgagaacgtgttttgcaccatgcagacctacagcaactccctcacgcttgtcatagtcacgtcgctgtttttattcacagctcagggaagtttatcgaatgccgtcgaaccaatcaaaaaacccctaaagctcgccaactaccgcgccacttgcgaaaaccgtacacgcacgctggttaccaggcttaacactagccatcacagcgtagtctggcaacgttatgatatctacagcagatacatgcgtcgtatgccgccactttgcatcattacagacgcctataaagaaaccacgcgtcagggtggcgcaactttcacgtgcacgcgccaaaatctcacgctgtacaatcttacggttaaagatacgggagtctaccttctacaggatcagtataccggcgatgtcgaagctttctacctcatcatccacccacgcagcttctgccgagccttggaaacgcgtcgatgcttttatccgggaccaggcagagtcggtgtggtcacggattcccaagaggcagaccgagcaattatctcggatttaaaacgccagtggtccggcctctcactccattgcgcctgggtttcgggactgatgatctttgttggcgcactggtcatctgctttctgcgatcgcaacgaatcggagaacaggacgttgaacatctgcggacggacctggatacggaacctttgttgttgacggtggacgggaatttggaataaaagatgcgtaacacctgtcgaagatgcgataactttacatacaggcaaacagtgtatacaattatagtattttgtatgttgcataaagttacatgcaacagtactgctaacagtactgcatccattacgctatccaacactgcctctaccacttttgtaaccaacatatattcaactccgaataacaacacatcaacgacgccacacacatctgtcacctcacaagcgtcaaccattggcaacatcaccaacgttacctccgacttgagtactttcacaaccgtatattctacattcaatacatcatttgccaatatatctaatacggctgtcactacagaattgatttcaacaaataccaacactatctcatcttttaccaacgtaacagcaaacgctacatcatcttataacacaacaatcaccgtaactgtcacgtcagatgaaacttcgcacaacgtatccactaataatgcacttataagcacaccatggcctacaaattgcagcgccacaacatacaccacgtacaaccttactaactcttccaacgcttgtcacacagagacaacaatcatacgtttcaaggaaaccaatacaacaggaatagaagggagtaatgtcaccataaagggtaattctacgtgggactgtctttcagtcgcctggatacgacattacaatagatccacacacggacatcatctaggttatcgtaagaacgcacatacccaatcttggtattggctacgcatccttacctctcacactgtatgtcattctcaacatgaaagaccttcactgtaccatgacttatgtcgttcgtgcaacaacacagaattacatctgtacgatctaaatatcaccaattccggcaggtacagcagacgttgttttaaagaaaattacttcacaggacatcacgaagatgaaaatttctacctattagtaacaccaaaaaatcatactgaagctattaatgctactttcgtttgccctagatacaacaccgatatcgaaaatgaagatagagagaaaggaagtcaacatactaacaatacacatcaccacaaacgtaatctctatcatagctcgcaaagaagccgcaccgtatggaccatcgtgttggtttgtatggcctgcatagttctgttttttgcacgacgagcctttaacaaaaagtatcatatgttacaagacaccgtcagtgaatcagaattcattgttcgatatcacccagaacatgaagattgagctacgtttccgggcagacatcttatgaagctgaacaataaactaaaacattctgtaagactcagcgttcaaaggaatattaatgcccattgagcgaaaactaatattgcaatggactggcgatttacggttacgtggaccgttacttgtgatggtttcaattatacagtccataaaagatgcgatcgcagttacgaggtaatcaacgtaacaggatacgttggtagcaacataactctaaaaaaatgcaatcagactgagaaatggcacaatgtagactggattcattatgagtaccccacgcataaaatgtgcgaattaggcaactatcaccaaaccacaccacggcacgacatatgttttgactgcaacgacacctccctaactatctacaacttaaccacaaaaaacgctggaaaatataccaggcgtcaccgtgataacggtcaagaagaaaattactacgtaacggtgttaattggagacacaacgttattcactcttggcacatgccctgtaagatataaagaatctacgaacactgaaaacaccattggaagtagcatcatagaaaccattgagaaagctaacattcccctgggaattcatgctgtatgggcaggcgtagtggtatcagtggcgcttatagcgttgtacatgggtagccatcgcattcccaaaaagccgcattacaccaaacttcccaaatatgatccagatgaattttggactaaggcttaacatgctgatcaataaactttttttaaccaataacatgtctccgtttttttttgttaacaacctatgatataaagcgttatattcagtcgttactaaacaaaaaaacatgggcatgcaatgcaacactaaattgttattgccagtcgcactaataccggttgcaatcatcctaattggtactctagtgccgatacttttacatgaacaaaaaaaggcgttttactggcgactttttctgcaaagtcaacatgtagaagcacccattacagtaacgcagggagacacagtctacctagacgctagcaataatccctgtaattattccagcttttggtaccacggtaattgcgaactttgtggatggaacggatatctacgcaatgttacacattactacacaaacacatcgtgttccccgcaattcatctgcataaacgaaactaaaggtctgcagttatataatgtaacattaaacgattcaggcgcttatactgaacacgtttacgaatgtgacctttcgtgtaacattactactaataacgaatatgaaatactcaattattttgataactgtaactacaccataaatagcaccaagcatattatcaccgtggtgtcttcacgtcattctaaacaaacaaattcccacgtatccactcacgctggttgggcagtcgccgtggtgacggtaattatgatctacgttctgatccactttaacgtcccggcaactctgagacacaaactacgaactagaaacaacgtaaatcgcatagcgtgattataaagtatcgacgctaatttctccaagataaaatttgattactccgtgcagttctcaaaaactgtaaggccccgcttttccactccgtcatgaaggatcgcaatagaatactgctatgtatcatctttatttgcattatgtgcctcatttgtatttactttaaacgtcgttgtgtttttactccgtctccagacaaagcagatctgcgagtggaatttccctcgttacccccgtgtattggcatacagtgcgctgcatgagaacacgcgtgacacatagcgtacccctggacggtacagtttatgataacgtaattcagggaaagtatacattcataccaacatgttatcacataacacacagattttctgcgtgttttataaaagagcgtctcgaagcagcttgagccacactacggtccagatgacgagcgtaattaaaaatatgccgcgcagtattcgaaagccgtactgagcgtgcgaggcgggtagggtgccgaacgacggatatgcgtcgttgtcatcttcgactataaggatcgcgaccgagtcttcggccatggtaaacgtcaccctgtgtggctggtatgtagcgtatccggtttggaattgttctgctccagctcgggggatagtgaggaattctcaagggatacgggacccaatgactggataagagaagggtttttccccgtaagatgatcctcgtatcacatgaggtctggatatgtataaatgaagagtgaaataggcacagggaatcagatgccagcctcgtgatgcagccgctggttctctcggcgaagaaactgtcgtctttgctgacttgcaaatacatcccgccttaagcgatgagtctataaagcaccgttgcccgagtacggtaaaagtgacccggattgtagaacgtcctttttttttgtttttgcatcgtttatcgtcactactagtgcaatattttgattgtaaggctgaaagagtatcgttatgatgcttagaacgtggagattattacagatggtactgcttgccgcgtactgttattatgtttttgcgacttgttcaatcagcacgacgactgctcctgtggaatggaagtctcccgaccgtcagattcccaagaatattacctgcgctaattactcagggaccgtcaacggcaacgttacatttcgaggtcttcagaacaaaacggaagactttttgtactggttgttaggatggggtcataagtccatttgttcgttcttcccgaaactccagggtaactatgacgaacaacattacagatatgaagtagcgaacctgacgtataactgcacctataaccgcttgacgttgctgaatctgacgacggaaaacagcggaaagtactatttcaaaagggaagatgcgaatttcaccttctattactcttgttacaacttgaccgtgtcctaaagatcgcacgtgaagtttcacagagccgcgtggctgtagctattgtgtttacgttgcttttgaaatgttaagcgtccctacggcgctaacatgtttctaggctactctgactgtgtagatcccggccttgctgtgtatcgtgtatctagatcacgcttaaagctcatgttgtcttttgtgtggttggtcggtttgcgtttctatgattgtgccgcgttcgagtcctgctgttacgacatcaccgaggcggagagtaacaaggctatatcaagggacgaagcagcattcacctccagcgtgagcacccgtacaccgtccctggcgatcgcgcctcctcctgaccgatcgatgctgttgtcgcgagaggaagaactcgttccgtggagtcgtctcatcatcactaagcagttctacggaggcctgattttccacaccacctgggtcaccggcttcgtcctgctaggactcttgacgcttttcgccagcctgtttcgcgtaccgcaatccatctgtcgtttctgcatagaccgtctccgggacatcgcccgtcctctgaaataccgctatcaacgtcttgtcgctaccgtgtagctagttagccagctgtgtgtagtgttttgcttttgcatatttgttttcagtcagagagtctgaaacggggtgggagggacttttgcgggtagtgcatgctaagatgaacgggtgggctggggtgtgcttgataactcactgtttgaatacgcgctcacgcacatatgtagcactcaacatgttagcttttgcccgcacgccccggggcgtgccgagctgcctttttaataaagtctgggtttccagatacgcgctggttctgattttgatggtttgtgcctctgaaagctctacgagctgggccgtgacatccaatggactgcctaactgtagcacggtaactagaacagcgggtcaagacgctgaattgcacggtccggcaccgttaagctgtaatgtgacccagtggggacgttacgagaatggaagcacacccgtgttatggtgcactttacggggatcaagcatgcgagtctcattaggacaccgtgtagcgtttggctgttcttggaaaacattttttatttataacgtttctgaaagtagcggtggcacttactatcaaaaaggttacaactgcaccgacaaacatataacactatcttgtttcaacttaacggtggttcctcgagcggttcaaagcacaaccaccgtaatgacacccacgctggttacaaactccacattcagtgtgtcacttgttccgttgagactgacgacaaattccagcgcgtttggacacgctatttatcaacgacaacagcgtgttgaaaacgggacgttatccaagaacataactaacttggcattcacctatggcagctggggcgttgcgatgctgctgtttgccgccgtgatggtgctcgttgatttgggtttgcctcaatcggcttggcgacgctggcgaagccacgtggacgatgaagaacgtggtttgttaatgtaggaaataaaaggcagtttgagcatgactgtttccaaaccgtaacgtggtaaataaatcatggcttccgacgtgggttctcatcctctgacggttacacgatttcgctgcagagtgcattatgtgtacaataaactgttgattttaactttgtttgcccccgtgattctggaatccgtcatctacgtgtccgggccacagggagggaacgttaccctggtatccaacttcacttcaaacatcagcgcacggtggttccgctgggacggcaacgatagccatctcatttgcttttacaaacgtggagagggtctttctacgccctatgtgggtttaagcctaagttgtgcggctaaccaaatcaccatcttcaacctcacgttgaacgactccggtcgttacggagcagaaggttttacgagaagcggcgaaaatgaaacgttcctgtggtataatttgaccgtgaaacccaaacctttggaaactactccagctagtaacgtaacaaccatcgtcacgacgacatcgacgatgatcgacgcgaaaagtaacgttacagggaacgccagtttagcaccacaattacgtgccgtcgctggattctccaatcagacgcctttggaaaacaacacgcacctggccttggtaggtgttgttgtgtttttagttctgatagttgtttgcattatggggtggtggaaattgttgtgtggtaaaccagagttatagtaatgtgctttttatcagggagaaggttttgtgccaacaatgactagcccgggactatctgcgtcagaaaattatgacggaaattatgaattcacggaaaccgccaatacaacgcgtacaaatagaagtgactggacaacgttagaaaccagtgcattgctattgaaaaacacggagactgcagtgaacctcagcaacgcgactacggtcatcccacaacctgtagaatacccggctggggaagtacaatatcaaagaacggcaacgcattattcttggatgctaatcattgtcatcattctcatcatttttattatcatctgtctacgagcacctcgaaaaatctaccatcactggaaagacagtaaacagtacggacaagtgtttatgacagacacggaactgtgacagtgatgtctaagcgtttgcaggtatttccatggataacaattttattttacacatcaaaatcccagtattggaactatatggcaataccatgtacccctacagttggatacggcagtcataatattagcttgcatccgcttaataactcattatttcaagacgatgtttttgaatggtacatagacaaaccaatggttacaagttatgtctttatcaaagtaatgaacgcacaaaatccaatctagactctccaaatattgtgtggcaatgcacagataatcgtacactaattctcatgaacttaaccacaacatacagtagaaactattattttcaatcctttaaatatctcggacgaggagtaccaaaaccgaataacttgtgttataacgttagtgtacactttacccaccaaacacattgccatacaactacatcatccctgtatccacctacatctgtacacgattcattagaaatatcacagtcattcacctcaaccaacttcacacataccgcggtccactacgccaccggtaacgttgaagcacaacacgacactaccactccacatacaatgtggatcatacccctagttatcgttataacaatcatcgttttaacttgtttcaaattcccccagaaagcttggaataaattcacacaatacagatacagcggtatgctcgccgccgcttaaagaatcaacgccaaggaaaccaaaacgtaaaaagaatagatatgtacgtttatttttcagctcactgtttgaataccgtaaacataatgacgtacatatacgtggttatacaacaggtgtttgtgttatgcggcgactgattaaccatatcgtgaaccatgatcttttccgatggtccgtcgtgaccgcaatgatattttacagatattccgaaacctgtatggaggtcactgtcagagtaggtgatccagttaccctcggtagtggacatggttatcatccaggtagggataacagggtaatgatcctctagagtcgacctgcaggcatgcaagcttgagtattctatagtctcacctaaatagcttgg

SEQ ID NO: 11 - DNA, 18036 bp, Cytomegalovirus HCMV
  misc_feature: HCMV fragment post-editing
acgacggccagtgaattgtaatacgactcactatagggcgaattcgagctcggtacccgattaccctgttatccctaccattccgggccgtgtgctgggtccccgaggggcgggggggtgtttttagcgggggggtgaaatttggagtcttggagccgcgtgtgctgtggaggacggtgacggtggtaagagtgtgctgcggtgcggttgggacggcggcggcgaataaaagcggcgtgcggcgcgcacggcgaaaagcagacgcgcgtctgtgttgtgtgtctttgaccgcggcggaacacacgcggaaaagcgagtcccaggggacacacgacgagcgagtcccagggggggacgacgacggccagggacgcggaaacgacgcggaaaagaggaagtccccagggggacgggcggaaaagaggaagcgcctaggggaccgcgggggcaggaacagacgaagtacgccgcaacccgcgtcgaggacacacgcagaagcggccgcccaggggagggggggggggggactcgcgggccccggggcacacttgttgttccctccggccgccgacacgcaccccgaagccgcgcacaccgccgacacacccctgacacacccgcgacacacccgccacacgcccgacacacgcccgcgacacacccgaccgacacaccctgacacaccccgccaacacacccagccgcacccgccccgccaacacacccccgacacacccgacacacgcccgcgacacacccggcacacacccacccacccagccgcgcccccgacacaccccgaacggcgccggtgcgggacagggctcacggaggtttgcgggccgtgagcacgcctccctttgtacacactaccggtgcgtggcgtcccacgctatttgttcgcgagaccggactaagggaggtttgcggtgcgtcagcgcggggcggcgtttgcggcgtgtttcgaccagcgctttgtgcgcgctgcctgtgcgtgtcgtcccatggtctttgtcagcggcacggcgctggggacggggtttcaccgcgctgagggatctttctgcgggtgtgagggacggagcttttttcgcacgctgggcaccgggctgggggacggggggtgtgcgggacggcggtggggccggggcgttgcgggtacggggattacgctgggaacggggactcgcggacccgggctgagggacgggggtggcgggggtgtttgcggcgaggacgggggccttttgcggcggggacggggactcaccctcgcctatttaacctccacccacttcaacacacacatgccgcacaatcatgccagccacagacacaaacagcacccacaccacgccgcttcacccagagtaccaacacacgttacccttacaccacagcaacacacaaccgcctatccaaacctcggacaaacacgccaacgaagaacaccgcacgcagatggagctcgacgccgcggattacgctgcttgcgcgcaggcccgccaacacctctacgctcaaacacaaccccaactacacgcataccccaacgccaaccctcaggaaagcgctcatttttccacagaaaatcaacatcaactcacgcatctacttcacaacattggcgaaggcgcagcgctcggctaccccgtcccccgcgcggaaatccgccgcggcggtggcgactgggccgacagcgcgagcgacttcgacgccgactgctggtgcatgtggggacgcttcggaaccatgggccgccaacctatcgtgaccttactgttggcgcgccaacgcgacggcctcgctgactggaacgtcgtacgctgccgcggcacaggctttcgcgcacacgattccgaggacggcgtctctgtctggcgtcagcacttggtttttttactcggaggccacggccgccgtgtacagttagaacgtccatccgcgggagaagcccaagctcgaggcctattgccacgcatccggatcacccccatctccacatctccacgcccaaaaccaccccagcccaccatatccaccgcatcgcacccacatgctacgactcgcccacatcacacgctctttcctatcccttctacaccctcagccacggttcacaatccccgaaactacgccgtccaacttcacgccgaaacgacccgcacatggcgctgggcacgacgcggtgaacgtggcgcgtggatgccggccgagacatttacatgtcccaaggataaacgtccctggtagacggggtagggggatctaccagcccagggatcgcgtatttcgccgccacgctgcttcaccgatatccaataaacccatcccctcgccacgacgtctccgcgtatctttgtagcctcaggaatccgtccccacgtccatccatcccgagcactccacacgctataacagaccacggacacggcaaatgcatgcaaacttctcatttattgtgtctactactctgtgttgctacagggagtgaagggggtgaaggcaaagaaaaaaaaaaggaacaaaataatagattagcagaaggaataatccgtgcgaccgagcttgtgcttcttttcttataaggaggcaaatatactagggaaaacttaagaataggaagaaaccgaggtttgggagaaaagctgagataaaatagcgcattttccatacagaggttgttgtttttgtggatcctaagaggtttcaagtgcgaatctcaaagttctcacgagaatattgtcttcaagaatcgacaactgtggtccaagatttttttttggtctttttaggttctgcgagggacatcacgatggatcgttgcgatgaagtcacgcgtacgcctctggtgtggcgcggtgtcgtgacaggagagtgtgttttcagtgcagagctgtcttgattcctatatccgagtatctgttttctcgtaaggacggtaatcttctttggtgtaagtacatctaaaagctgcaaactatattttaagggctgtctctaggtgtactttgatgctggagtttttcgctgtgttgatgtgaataaatctactactactattatatgcagaaagagtgattatgccgagacaagattgcattggctgaactgtttcaaaaacgcctacactctacttatccgtaaacctaaggtaatactatgtgtaagttgtttttttttctttttgtagtaaaatggtgatacgtgcaattaaaactgtattccatgtttccatcctttcatttcaactttaaaggcggctttgagagcgaagaagtgcgaggataaaaatggatgactccttcgtgtccagggagtcgactactgcaacgctgattgattaaaagatggtctccgatgatgatgttgttattgatcgaatcatggtgcagaacggcgacggagaggagcgtgtccgccgccgggaaggtggtctctttctcttttcttttttcaagaaatcttccatgtgtttatcgtagtgatcgaaatcgactgatctcgggttctttttgttggtttcttttcggttaatcatgtattgttttctttttttacagaaagatacttttttcatgagcaattcctcgcccggcgccggcatgccgaggtggggccactgcgatcagcggcatgccgacgccgacccggggatcttggattcaccgttttctctcttctctctctacatacagaccgggtggcaggagcggtaaggaatcatcgtcgtctttcattcttcgatgattatggtaatactaaatcttatctaggagcatatacatctaagattggagtactagtagtcgtttgtggtttctattttttttatatttatctatgacagtttttctgtttttcgttttgataataatataataaaaactcatggacgtgaaatctggcttggttgtggtgatttcattctcattattgttgttttctttccgtcttgcggatgaagatgttgcgatgcggttgttgttggtgttgctatacaccgagagagatgatctttttgttcttctggttcatttcctatgattgtttggctgctgaccgacgcgtcaggatgtgcagggcatgcggggaatcaggaccggacacgggataatttcatctacctatacggagatcgcggtcctcgccatgaggatcgcgacaggcgcgtcgagggggcaggaacacccttgcggattgacattcttggtggtgtttcgttgttgtcggtagttgttgttgacgatgaggataaataaaaatgaccttgtttttgttctgttttctcttgttgggaatcgtcgactttgaattcttcgagttatcggaaagctgaggtacccaaatgtctgtagcttttttctttttaccctcttgtttatcatctgcgattcgtggtaggtaggagagggaaatgataatccgagattaaggaaaggagaagataaaaaataaaaaaaaaataataaaacagaagccgaccggccgccgacccgttccccaggaccagcctacgaggaatggataacgcggtggcgacggcagcggtggtggcgctgggggtggcggcagtggtactgctgatggtagtcgggacggaggagaggcgatgcatacatacacgcgtgcatgctgcatgggtggatggtacggccgggagacgcggaagagaaactcacataaaaaggtgacaaaaagagcggttgaaaaaagaaaacgagattcgaccagacagaagagaaggaccggggcttggcgacccttccacgactgctgttgtcatctcggctcccccgtcttctcccggccacgggcggctaagtcaccgccgttctccccatccgtccgagcgccgaccgaccagccggccgattcgcccgccggggcttctggagaacgccggggcagcagcgatctggggaagccgctaaacccctgcgtttttatatggtagctctgccgagcgcgggctgacgcgttgagtaagcggaaagacgtgtgtgacgaaaaggggtcccatggtatttcacgtgacgatgaggagatgcggtttggagcacatacggtttagaaaaagggagttgtcgtgacaagggctgagggacctctgtctccatgtgtgtataaaaagcaaggcacgttcataatgtaaaaaagaacacgttgtaaacaagctattgctgtatcattcggctgactatgcttcattcggactgattttcttttcctaacggcgtaacttaaagtgattaacgtatgatatttgttccccagagttatactatagtcatcatcctaaaattcagatataaatgaacacatgtcgtatgggattattaagaaaccgaaactctccacagttcaccatcttcttcgtcattcaaccgatgacccactccgtacaacgaatcagtctgctgtgtcacactgcaaactactagcgacgtatgcaaacaacttgaaacacgggctgttgtattgacgaccgttgtaccattactagtcacattgcatagagaccatccaccgtcatcccatctttcccacccgatggaaaaccgtcttctatcatcaactatggtaagatttcgaccctgcgaggtattcagtttccccatatccataacctggattttatcattaaaccccaatattaaacacttttttagtacccccccacccaccaaaaaatgtgactggaccggttcctagcagctctgggagccatgttcaggttgaaccacagctacagcgaaaccgagtccagtgaccggtaaccacgtccagcccctgcgtatgtaccagtccaagcacgtccggtcattgttctacacaggaaatctaactaggtcaacgcaattttattccaccgttacgcagaatactaacaaacaaacacacaaatttaacgaattacacgtagtttattacatgaaaactgtaagaacaccaattcactaagcgatacaacatttagctgacttccaagtgccacacatcaccactgtattcatccatgttttcaccgaaccaacgagacagatcgaagaagccagaatctcccgactttaaattacataaatccaacgtattatgaccacagctcgacacacaaatagttgcgttactattcacagtagcattacctatacccgtaacgttgcacaaccactgatcaccattgttaccaaaaacggttttccacttagttgtcaacggatctttcccatgcgtaatggtcaaattactaccagtcgtcgcttttagctcattacgagtattatccgcatccacatatatcaacgtcatagctaggcacgctataagtaccccccccccacaatggaatgttgccaaaccggttctttcccgttatagccatagcgttcccaggcaaaagcaaacgccaaacctaatgcagtgaaaagcgcttgcagccagaaccagcttatgtaccagccacaatcacatccggttattgtttccacaggaaatcctaccaggcaaagccccgcttgttttgttcctgaccatcttgtttagcaattcgtaaactgtcagcctagcgacgtccgtttagatcaaaagtcacgtatatagcgacgctgtttccacccgtttccccgtcccgccgtttccgaacaacccacccgggttcagacaaccgaccaccaacagaaatatacacacagaccaccgggagttcagttaaagatttcatcaggtttattttggctgctgctagtcttttgcttcttagaaaaaaaatacccatatagagaaataatgatagtttgacaacacatatggcagggatttcttcttcatcaataagatatgcaattcccccagggagagactttcaacaattgaatttacaaaaacaaaattacatcaggagaaagagaggatacattaataaatatattatatctggtgtatatactgaatgctgctggttcataaggtaacgatgctactttttttaattccaagatggtttttctttgttagtcttttgttgacttgctggttcctaaaagttcgcaaaaacgattgtgtgaagattatgacgttggttgactagttcatgagattctgctgtacgtgtgatggttattcgctggttcgttctaagatgagtatcgtactgtgtctgcgatggtcgtctcttactggcattctctcggctgcctcttgttttcatgattgaaaaggaaaaaaggactccgagggcgcggtcatcttttacttttcggttttctcgttggcgggtcagaggtagtcagatcatgagactgtcgtggtcgatgaaactgtgtctgctcaagtgacgtccatttcttgtacggagaaaaaagtcatcgggataaataaggctatacaaggcgttgtcaagcgtgcggctctaaacaaattaagcgatacaaaattacagtgatacgaataataaattaccccctccccctgtggtccccccgaggcgagagccacccatcgtgtactctcgcaccacccacgaccacagggggagacgggacgaagagacgacgcagagcgccatctcctcctggaggccggcggcgttaactgctacagctgcggcggcgacgacagctgcgatttgtcggccgacatgccgatggtatgggcggcggcggcggtggccgcggcagcggggaggagaggagagagaagaggagcggggcgtccgaaggcgaggatggcatggtctcgccggagcgcccggcttttatggaacactcgcgtccggttgggtatcacccacaggaagatgaatcacaacttccaaaccatcttgagacccgagtaacggtttacaggtcgcacgccagtctcagctaaaaacagcggacagtcccacgctgtttctgttgtggctctctccagtttcctcatcgccgtcttggtctccgtcatcatcggaagaataccacccgctctcatgcggcagtcgatcagcctcgatgaacgagacgcggcgacgcctttctacggccgactggttgtggtggtgaaagaagagcaccagcaatcccaggaggagcaacaagccctcacatgtccaggaggtcggggagagggcctgtcggagatgaccgtgaggcatcacgtacggcagctgaggagaaacggagaagaaaggaaaattaccgtcaggggccggggttcttattagagaaacagcacgtaggtcaggatccagatgctaatggcaatcatgatgacgatgatcatgcaggccaagacgcggcgcaccaatgcagaatccaatagccgccgtgcctccggttggtggccggcggcatctagagacatgatttgggggggggaccggcggcgcaaaaagacagggagatggacagtgccacggtgttttgttatgattaggacatggggaccggaagccgagacagagtactacagggtgttgaagggtaacgtgagggagatcatgtcatgggcgggctgaagaccgtgcggggaggatcgacgtgtgcggtgcttgtggaacacggtgttttaatatgtatccgcgtgtaatgcacgcggtgtgctttttagcactcggcttgataagctacgtgaccgtctgcgctgaaaccatggtcgccaccaactgtctcgtgaaaacagaaaatacccacctagcatgtaagtgcaatccgaatagtacatctaccaatggcagcaagtgccacgcgatgtgcaaatgccgggtcacagaacccattaccatgctaggcgcatactcggcctggggcgcgggctcgttcgtggccacgctgatagtcctgctggtggtcttcttcgtaatttacgcgcgcgaggaggagaaaaacaacacgggcaccgaggtagatcaatgtctggcctatcggagcctgacacgcaaaaagctggaacaacacgcggctaaaaagcagaacatctacgaacggattccataccgaccctccagacagaaagataactccccgttgatcgaaccgacgggcacagacgacgaagaggacgaggacgacgacgtttaacgaggaagacgagaacgtgttttgcaccatgcagacctacagcaactccctcacgcttgtcatagtcacgtcgctgtttttattcacagctcagggaagtttatcgaatgccgtcgaaccaatcaaaaaacccctaaagctcgccaactaccgcgccacttgcgaaaaccgtacacgcacgctggttaccaggcttaacactagccatcacagcgtagtctggcaacgttatgatatctacagcagatacatgcgtcgtatgccgccactttgcatcattacagacgcctataaagaaaccacgcgtcagggtggcgcaactttcacgtgcacgcgccaaaatctcacgctgtacaatcttacggttaaagatacgggagtctaccttctacaggatcagtataccggcgatgtcgaagctttctacctcatcatccacccacgcagcttctgccgagccttggaaacgcgtcgatgcttttatccgggaccaggcagagtcggtgtggtcacggattcccaagaggcagaccgagcaattatctcggatttaaaacgccagtggtccggcctctcactccattgcgcctgggtttcgggactgatgatctttgttggcgcactggtcatctgctttctgcgatcgcaacgaatcggagaacaggacgttgaacatctgcggacggacctggatacggaacctttgttgttgacggtggacgggaatttggaataaaagatgcgtaacacctgtcgaagatgcgataactttacatacaggcaaacagtgtatacaattatagtattttgtatgttgcataaagttacatgcaacagtactgctaacagtactgcatccattacgctatccaacactgcctctaccacttttgtaaccaacatatattcaactccgaataacaacacatcaacgacgccacacacatctgtcacctcacaagcgtcaaccattggcaacatcaccaacgttacctccgacttgagtactttcacaaccgtatattctacattcaatacatcatttgccaatatatctaatacggctgtcactacagaattgatttcaacaaataccaacactatctcatcttttaccaacgtaacagcaaacgctacatcatcttataacacaacaatcaccgtaactgtcacgtcagatgaaacttcgcacaacgtatccactaataatgcacttataagcacaccatggcctacaaattgcagcgccacaacatacaccacgtacaaccttactaactcttccaacgcttgtcacacagagacaacaatcatacgtttcaaggaaaccaatacaacaggaatagaagggagtaatgtcaccataaagggtaattctacgtgggactgtctttcagtcgcctggatacgacattacaatagatccacacacggacatcatctaggttatcgtaagaacgcacatacccaatcttggtattggctacgcatccttacctctcacactgtatgtcattctcaacatgaaagaccttcactgtaccatgacttatgtcgttcgtgcaacaacacagaattacatctgtacgatctaaatatcaccaattccggcaggtacagcagacgttgttttaaagaaaattacttcacaggacatcacgaagatgaaaatttctacctattagtaacaccaaaaaatcatactgaagctattaatgctactttcgtttgccctagatacaacaccgatatcgaaaatgaagatagagagaaaggaagtcaacatactaacaatacacatcaccacaaacgtaatctctatcatagctcgcaaagaagccgcaccgtatggaccatcgtgttggtttgtatggcctgcatagttctgttttttgcacgacgagcctttaacaaaaagtatcatatgttacaagacaccgtcagtgaatcagaattcattgttcgatatcacccagaacatgaagattgagctacgtttccgggcagacatcttatgaagctgaacaataaactaaaacattctgtaagactcagcgttcaaaggaatattaatgcccattgagcgaaaactaatattgcaatggactggcgatttacggttacgtggacgatactaatgtccgcgttgtcagaaagctgcaatcaaacctgttcttgtcaatgtccctgtagtactaccgttaactattcaactagtactgagacagccacatcaacatacagtacaacagttatcagcaataaaagcacttcagaatctataaattgctctactgcaactacaccagcaaacaccgtttctacaaaaccgtcggaaacaaccacacagatatccacaacgacgaacacaaacgttgagactaccacatgtaccaacaccaccacgaccgttacttgtgatggtttcaattatacagtccataaaagatgcgatcgcagttacgaggtaatcaacgtaacaggatacgttggtagcaacataactctaaaaaaatgcaatcagactgagaaatggcacaatgtagactggattcattatgagtaccccacgcataaaatgtgcgaattaggcaactatcaccaaaccacaccacggcacgacatatgttttgactgcaacgacacctccctaactatctacaacttaaccacaaaaaacgctggaaaatataccaggcgtcaccgtgataacggtcaagaagaaaattactacgtaacggtgttaattggagacacaacgttattcactcttggcacatgccctgtaagatataaagaatctacgaacactgaaaacaccattggaagtagcatcatagaaaccattgagaaagctaacattcccctgggaattcatgctgtatgggcaggcgtagtggtatcagtggcgcttatagcgttgtacatgggtagccatcgcattcccaaaaagccgcattacaccaaacttcccaaatatgatccagatgaattttggactaaggcttaacatgctgatcaataaactttttttaaccaataacatgtctccgtttttttttgttaacaacctatgatataaagcgttatattcagtcgttactaaacaaaaaaacatgggcatgcaatgcaacactaaattgttattgccagtcgcactaataccggttgcaatcatcctaattggtactctagtgccgatacttttacatgaacaaaaaaaggcgttttactggcgactttttctgcaaagtcaacatgtagaagcacccattacagtaacgcagggagacacagtctacctagacgctagcaataatccctgtaattattccagcttttggtaccacggtaattgcgaactttgtggatggaacggatatctacgcaatgttacacattactacacaaacacatcgtgttccccgcaattcatctgcataaacgaaactaaaggtctgcagttatataatgtaacattaaacgattcaggcgcttatactgaacacgtttacgaatgtgacctttcgtgtaacattactactaataacgaatatgaaatactcaattattttgataactgtaactacaccataaatagcaccaagcatattatcaccgtggtgtcttcacgtcattctaaacaaacaaattcccacgtatccactcacgctggttgggcagtcgccgtggtgacggtaattatgatctacgttctgatccactttaacgtcccggcaactctgagacacaaactacgaactagaaacaacgtaaatcgcatagcgtgattataaagtatcgacgctaatttctccaagataaaatttgattactccgtgcagttctcaaaaactgtaaggccccgcttttccactccgtcatgaaggatcgcaatagaatactgctatgtatcatctttatttgcattatgtgcctcatttgtatttactttaaacgtcgttgtgtttttactccgtctccagacaaagcagatctgcgagtggaatttccctcgttacccccgtgtattggcatacagtgcgctgcatgagaacacgcgtgacacatagcgtacccctggacggtacagtttatgataacgtaattcagggaaagtatacattcataccaacatgttatcacataacacacagattttctgcgtgttttataaaagagcgtctcgaagcagcttgagccacactacggtccagatgacgagcgtaattaaaaatatgccgcgcagtattcgaaagccgtactgagcgtgcgaggcgggtagggtgccgaacgacggatatgcgtcgttgtcatcttcgactataaggatcgcgaccgagtcttcggccatggtaaacgtcaccctgtgtggctggtatgtagcgtatccggtttggaattgttctgctccagctcgggggatagtgaggaattctcaagggatacgggacccaatgactggataagagaagggtttttccccgtaagatgatcctcgtatcacatgaggtctggatatgtataaatgaagagtgaaataggcacagggaatcagatgccagcctcgtgatgcagccgctggttctctcggcgaagaaactgtcgtctttgctgacttgcaaatacatcccgccttaagcgatgagtctataaagcaccgttgcccgagtacggtaaaagtgacccggattgtagaacgtcctttttttttgtttttgcatcgtttatcgtcactactagtgcaatattttgattgtaaggctgaaagagtatcgttatgatgcttagaacgtggagattattacagatggtactgcttgccgcgtactgttattatgtttttgcgacttgttcaatcagcacgacgactgctcctgtggaatggaagtctcccgaccgtcagattcccaagaatattacctgcgctaattactcagggaccgtcaacggcaacgttacatttcgaggtcttcagaacaaaacggaagactttttgtactggttgttaggatggggtcataagtccatttgttcgttcttcccgaaactccagggtaactatgacgaacaacattacagatatgaagtagcgaacctgacgtataactgcacctataaccgcttgacgttgctgaatctgacgacggaaaacagcggaaagtactatttcaaaagggaagatgcgaatttcaccttctattactcttgttacaacttgaccgtgtcctaaagatcgcacgtgaagtttcacagagccgcgtggctgtagctattgtgtttacgttgcttttgaaatgttaagcgtccctacggcgctaacatgtttctaggctactctgactgtgtagatcccggccttgctgtgtatcgtgtatctagatcacgcttaaagctcatgttgtcttttgtgtggttggtcggtttgcgtttctatgattgtgccgcgttcgagtcctgctgttacgacatcaccgaggcggagagtaacaaggctatatcaagggacgaagcagcattcacctccagcgtgagcacccgtacaccgtccctggcgatcgcgcctcctcctgaccgatcgatgctgttgtcgcgagaggaagaactcgttccgtggagtcgtctcatcatcactaagcagttctacggaggcctgattttccacaccacctgggtcaccggcttcgtcctgctaggactcttgacgcttttcgccagcctgtttcgcgtaccgcaatccatctgtcgtttctgcatagaccgtctccgggacatcgcccgtcctctgaaataccgctatcaacgtcttgtcgctaccgtgtagctagttagccagctgtgtgtagtgttttgcttttgcatatttgttttcagtcagagagtctgaaacggggtgggagggacttttgcgggtagtgcatgctaagatgaacgggtgggctggggtgtgcttgataactcactgtttgaatacgcgctcacgcacatatgtagcactcaacatgttagcttttgcccgcacgccccggggcgtgccgagctgcctttttaataaagtctgggtttccagatacgcgctggttctgattttgatggtttgtgcctctgaaagctctacgagctgggccgtgacatccaatggactgcctaactgtagcacggtaactagaacagcgggtcaagacgctgaattgcacggtccggcaccgttaagctgtaatgtgacccagtggggacgttacgagaatggaagcacacccgtgttatggtgcactttacggggatcaagcatgcgagtctcattaggacaccgtgtagcgtttggctgttcttggaaaacattttttatttataacgtttctgaaagtagcggtggcacttactatcaaaaaggttacaactgcaccgacaaacatataacactatcttgtttcaacttaacggtggttcctcgagcggttcaaagcacaaccaccgtaatgacacccacgctggttacaaactccacattcagtgtgtcacttgttccgttgagactgacgacaaattccagcgcgtttggacacgctatttatcaacgacaacagcgtgttgaaaacgggacgttatccaagaacataactaacttggcattcacctatggcagctggggcgttgcgatgctgctgtttgccgccgtgatggtgctcgttgatttgggtttgcctcaatcggcttggcgacgctggcgaagccacgtggacgatgaagaacgtggtttgttaatgtaggaaataaaaggcagtttgagcatgactgtttccaaaccgtaacgtggtaaataaatcatggcttccgacgtgggttctcatcctctgacggttacacgatttcgctgcagagtgcattatgtgtacaataaactgttgattttaactttgtttgcccccgtgattctggaatccgtcatctacgtgtccgggccacagggagggaacgttaccctggtatccaacttcacttcaaacatcagcgcacggtggttccgctgggacggcaacgatagccatctcatttgcttttacaaacgtggagagggtctttctacgccctatgtgggtttaagcctaagttgtgcggctaaccaaatcaccatcttcaacctcacgttgaacgactccggtcgttacggagcagaaggttttacgagaagcggcgaaaatgaaacgttcctgtggtataatttgaccgtgaaacccaaacctttggaaactactccagctagtaacgtaacaaccatcgtcacgacgacatcgacgatgatcgacgcgaaaagtaacgttacagggaacgccagtttagcaccacaattacgtgccgtcgctggattctccaatcagacgcctttggaaaacaacacgcacctggccttggtaggtgttgttgtgtttttagttctgatagttgtttgcattatggggtggtggaaattgttgtgtggtaaaccagagttatagtaatgtgctttttatcagggagaaggttttgtgccaacaatgactagcccgggactatctgcgtcagaaaattatgacggaaattatgaattcacggaaaccgccaatacaacgcgtacaaatagaagtgactggacaacgttagaaaccagtgcattgctattgaaaaacacggagactgcagtgaacctcagcaacgcgactacggtcatcccacaacctgtagaatacccggctggggaagtacaatatcaaagaacggcaacgcattattcttggatgctaatcattgtcatcattctcatcatttttattatcatctgtctacgagcacctcgaaaaatctaccatcactggaaagacagtaaacagtacggacaagtgtttatgacagacacggaactgtgacagtgatgtctaagcgtttgcaggtatttccatggataacaattttattttacacatcaaaatcccagtattggaactatatggcaataccatgtacccctacagttggatacggcagtcataatattagcttgcatccgcttaataactcattatttcaagacgatgtttttgaatggtacatagacaaaccaatggttacaagttatgtctttatcaaagtaatgaacgcacaaaatccaatctagactctccaaatattgtgtggcaatgcacagataatcgtacactaattctcatgaacttaaccacaacatacagtagaaactattattttcaatcctttaaatatctcggacgaggagtaccaaaaccgaataacttgtgttataacgttagtgtacactttacccaccaaacacattgccatacaactacatcatccctgtatccacctacatctgtacacgattcattagaaatatcacagtcattcacctcaaccaacttcacacataccgcggtccactacgccaccggtaacgttgaagcacaacacgacactaccactccacatacaatgtggatcatacccctagttatcgttataacaatcatcgttttaacttgtttcaaattcccccagaaagcttggaataaattcacacaatacagatacagcggtatgctcgccgccgcttaaagaatcaacgccaaggaaaccaaaacgtaaaaagaatagatatgtacgtttatttttcagctcactgtttgaataccgtaaacataatgacgtacatatacgtggttatacaacaggtgtttgtgttatgcggcgactgattaaccatatcgtgaaccatgatcttttccgatggtccgtcgtgaccgcaatgatattttacagatattccgaaacctgtatggaggtcactgtcagagtaggtgatccagttaccctcggtagtggacatggttatcatccaggtagggataacagggtaatgatcctctagagtcgacctgcaggcatgcaagcttgagtattctatagtctcacctaaatagcttgg

SEQ ID NO: 12 - DNA, 2310 bp, LKA1 gp49 sequence
atggcgcaaacacccagtacatgggccgactacgtaggcgacggcgtagaggatacgttccaagtcacattcccgtaccagaagcagcaagaggtgtttgtgactgtgggcggcgatccggcagctttcacattcatctcggcaggttggattcaactggcagcggtcccggtaaatggggccgcaatccgtgtacggcgcagcactgaggcattcgagcctcggcacgagttcgccaacggcgtgccattactgccgcgattcatagacgagaataatacccagttcttgtacactgtacaagaggcagtgaatgagacacatggcattgcttccgaagcgctgagtgtcgcagaggaggccagaggcattgcgcaggcggcatcggataaagtggatgctgccaccattgactccgcacaccagttgcgtctagacctcgccgacccggcgaaggggcctgggctgctaggctacgaccgagacgtaagttatccggtcgggtcggtcggtcaaagcctacagtttctggaaatgggtcgggtcacaccagcgcaatttggcgccgttggtgatggcgccagccaccccctctctgagcgatacgcaactctagcggaagctcagactgtctatccgcatgcagtcgcactctccgacgaaatagactgggccgcattgcaagctgccgtggattcaggggcacctgtacacataccgtctggggactatcagataaatagggggattagcagtacgggctctctacagattgcgggtgatggcgctacatctattatacgcccgactgctgcgttcactggtacatcggtcctcagttgtgtggggagcttagttgccttgccgaatatatcctccgtgtcggctgggtccctaaccattgactttgccagcacccctaatcttgtagcgggggatgtattcatcatctacaacccgactgatagcagcttctcgggatttcggacgagctatcgcgcaggagagttctgtgaggtcagggcggtttctgggaacaccgtgacaatccgttccgcactctatgccgcatacgacggggctactgttgctatttacaaagtagtctctggtgtagttgatatagctagcatccaaatcgttggcgggacagtcccaatgaatggactgttagtggaggctgtcgtttcaccgcgcgtcgatgacgtgacggtcacccttgcaaacaacgccggtgtgtattttgcccgctgctatgacgctaagatcacaaacagtaatatatcgaacatcggcgacggtggcgatgactatggaatcatctttgggaactgtcacgacggtggggcagacaactgtaaagtctacgctaggcgacatgccatcgccacgggcggcgatgcagaagtaggctgcgttccggtccgtaatgtgcgtatgcgtaactgcacacttaggaatgatattacctctggtacacactgcgcagacttccacggtaacgccgaggattgcagctacgaaaactgcacaatctacggtggtgcaacttggcaggggaaggatatcagctacagacactgtacaatcactaacgcgtcgggtggttggattgttatatccgctgagattcttggtggtacattccttctcgaccaatgcacattgtacacaaccggcgatccgcagcctggtaaccgtggggttatagatgtaggtgggaactccgcagtcctcactacaaatacaacgcaaccctgtaacttccttatacaaggcggcagtctgcgagcgcccagcttaagtacgtctagttacctactgcgcgcacgtcttgagggtagtacagttccagtaaacatacagtacagcggacaggctattgatgtaggctctctgggcaaggtactacaactcgatattacctcgggcagtacctctcctgagtatttgatcgtggagaatttagcggggttgccatctggcatcacgctggcgtctgctgctggtggtttcgcaagtgccccgatgcgtatgcctgtgctgggtggtagggttcaagtaactacggcaaccaacgcgagtagcgttactgctccagtaacgttcaggtacatttatcctaaggccccaaccgtccaggtcacaaagacggacaggagctacgccggtaacagggtcggcgttgctatcgccaatccgacctctgcgtctggggcgacgttgggtctgttcacggacgacgggacaaactttagctcagccgttactaaccagttgaactggcaggcaggtatttatgaggtgtaa

SEQ ID NO: 13 - DNA, 1956 bp, Phikmvlikevirus NTUH-K2044-K1-1
  misc_feature: NTUH-K2044-K1-1 gp34
atggccctgatccggctcgtggcgcccgagcgcgtgttcagcgacctggccagcatggtcgcctatccgaacttccaggtgcaggacaagatcaccctgctgggctcggccggcggcgacttcaccttcaccaccaccgcgtcggtggtggacaacggcaccgtgttcgccgtgcccggcggctatctcctgcggaagttcgtcggcccggcgtatagctcgtggttcagcaactggaccgggatcgtcacgttcatgagcgcgccgaaccggcacctggtggtggacaccgtgctgcaggccacgagcgtgctgaacatcaagagcaacagcacgctggaattcacggacacgggccgcatcctgcccgacgccgccgtggcccgccaggtgctgaacatcaccggctccgcgccctcggtgttcgtgcccctcgccgccgacgccgccgcggggtcgaaggtgatcaccgtggccgccggcgcgctgtccgcggtgaaaggcacctacctctatctgcgctccaacaagctgtgcgacggcgggccgaacacctatggcgtcaagatcagccaaatccgtaaggtggtcggcgtgagcaccagcgggggcgtgacgtccatccgcctcgacaaagccctgcactataactactacctctcggatgccgccgaagtgggcatcccgaccatggtggagaacgtcaccctggtgagcccgtacatcaacgagttcggctacgacgacctgaaccgcttcttcaccagcggcatctccgcgaacttcgcggccgacctgcacatccaggacggcgtcatcatcggcaacaagcgtccgggcgcctccgacatcgagggccgcagcgccatcaagttcaacaactgcgtggatagcaccgtgaagggcacctgcttctataatatcggctggtacggcgtggaggtcctcggctgctcggaggacaccgaggtgcacgacatccacgccatggacgtgcgccatgccatctccctgaactggcaaagcaccgccgacggcgataagtggggcgaaccgatcgagttcctgggcgtgaactgtgaggcgtacagcaccacccaggccggcttcgacacccacgacatcgggaagcgtgtcaaattcgtccgctgcgtgtcctacgacagcgcggatgacggcttccaggcccgcaccaacggcgtggagtacctcaactgccgcgcctaccgcgccgccatggacggcttcgcctcgaacacgggcgtcgccttcccgatctaccgcgaatgcctggcctacgacaacgtgcgcagcgggttcaactgcagctacggcggcgggtatgtgtacgactgcgaggcgcacggcagccagaacggcgtccgcatcaacggcggccgggtcaaaggcgggcgctacacccgcaactcgtcgagccacatcttcgtgacgaaagatgtggcggaaaccgcccaaaccagcctcgagatcgacggcgtctccatgcggtacgacggcaccggccgcgccgtgtacttccacggcaccgtgggcatcgatccgacgctcgtgagcatgtccaacaacgacatgaccggccacggcctgttctgggccctgctgtccggctataccgtgcagccgaccccgccgcgcatgtcgcgcaacctgctcgacgataccggcatccgcggcgtcgcgaccctggtcgcgggcgaagcgaccgtcaatgcccgcgtccgcgggaacttcggcagcgtggccaacagcttcaagtgggtgtcggaggtgaagctgacgcgcctcacgttcccgtcgtcggccggcgccctcacggtcaccagcgtcgcccaaaaccaggacgtgccgacccccaacccggacctgaacagcttcgtcatccgcagcagcaacgccgccgacgtgtcccaagtcgcctgggaggtctacctgtga

SEQ ID NO: 14 - DNA, 2184 bp, T7-like Pp15
  misc_feature: Pp15 gp44 sequence added
atggcacgaactatcgtccagaacgccctaacaggcggacaacaggacttcgaggtacctttcgactacatcttgcagcgcttcgttaagcttaccctgatcggtgacggtaaccgacaagagctggtcctcggtaccgacttccggttcatcggtcctcgcaccgttcgcactaacgtcttctggggaccagcgcaggggtatacctccatcgagatccgacgagttaccagcgcttctgatcgtcgcgtagagttctcggacgggtccatcctgaccgcaggtgatctgaacatcgcccagcttcaggccatccacattgccgaagaagcgcgagactctgccactgagaacctgagcccagatgctgatggcaactacgatgcacgtggtgcgcgcatttacaacctcggtgacgctgttcagccgaaggatgcggtcaaccggtacactcttgacctcgctatcgcagccgctctggccatgaataccggcaacccgaacaacgcccagaacatctcgtacacccctaacgggcctggtcagtcgatccgaagtgttgaaggccgtctgcgggatgctgtgttcgtctcggactacatgaccactccacgtgatggagttaccagtaaccagcaggacctcgaaaaggcactcgctgcggcgaacgctaaaggtgccgacctattctggcctgacgacatcccgttcttctccacgtccccgctggcactgatccacgcggtctaccatgttggacgtggtgtcatcaacgcgaacggtacgctgttctacgtgaacccgaagaacggccaacacaacaggctacacgtgtctcccgggggcaccggggatggtctggcagctggccgcccactggggaccatctggagtgcactcgcggcccttaacatgcgagccccactgaccacgcgctggtccttggagatgaccgctggcgcctataatgaagccgttacacttccgaactacctgaccagctgtaacgactacttggcgtttaactggccgaacaccggtcaggaacgtatggagcccactgcgtacccatcagctctcgacggcacaggccagaccggcctcacaggtttccacactggcatcggcaaccgcattaccatcaacaacgtgtgcatgtccaactggtacgacactgcgctgactcctacccaacaggtgcgaagagcgttcgttgtaggtgcgtattcgactgcctacgtggtcaactgcgcgttcatttacaacggcatcgcgagcgtgtctgtgctgcccggtggcactgctatcgtaaccggtggcatcgtcgatggtgggcggttcggcctcgacaacactggcggtcgcctgtccctgacggcaaccaagagcaattatacgcaggtccggaactgcctcgaatatggactgtactcgaagcatgacgcatcgaccgtaatggacaacaccgagttccgcaactgcggtaatcaccctgcggctgttgcgtatggtgctgcaatcttcgcgtacaagttcaactgttctgttgacactcgtggggtcaagttctacggcaacaacatcgcccagcactgccgtggcggtatcacctcggacaatccgggcgatccggacatctacggtaccggcgcagatgctaataagcgtctattcctgtgcaccggtggtggctctgacgacatccagttctacgaagctcggcgcgtcatggacatcacgaagcgcactggtggcggctcaactactgccagcgtatcgtcgctgctactggctgccgttgcgtctgtccgtaagggctactttgcgcacaacgatcaggtgatccggatgaccctgatgttccgcgctacaggctcggctggcatcttcacgccgaccttgcgcacacctctggggactatccctctgggtagcttcagggtcgcatcgggacagtacggcgagatcaagttgaccattcgacctactctgacatctgatggtctcatagtcgggttctcctgcatcaacgccgtgcagaatcttgggtcctctgttggtcaaatcatcgtcagcggcaccgtagacctccgcaccgtcgaccagctggtcgagatgtggggctattcggaagctggtggcaccgcttcgtacattcaaggcctgatcgagctggtcgggtga

SEQ ID NO: 15 - DNA, 1089 bp, Aggregatibacter actinomycetemcomitans
  misc_feature: dspB sequence added
atgaactgttgcgtcaagggcaattccatctacccccagaagacctccaccaagcagaccggcctgatgctcgatatcgcccggcatttctacagccccgaggtgatcaagagcttcatcgatacgatcagcctgagcggcggcaacttcctccacctgcacttctcggaccatgaaaactatgccatcgagtcgcacctgctcaaccagcgggcggagaacgccgtccaggggaaggatggcatctacatcaatccgtacaccgggaaaccgttcctgagctaccgccagctggacgacatcaaggcctacgccaaggccaagggcatcgaactgatcccggagctggacagcccgaaccatatgacggccatcttcaaactggtccagaaggaccgcggcgtcaagtacctgcaggggctgaaatcccgccaggtggacgacgagatcgacatcaccaacgccgatagcatcaccttcatgcagagcctgatgagcgaggtcatcgatatcttcggcgacacgagccagcacttccacatcggcggcgacgaattcggctactccgtcgagagcaaccacgagttcatcacctacgccaacaagctgtcgtacttcctggagaagaaggggctcaagacccgcatgtggaacgacggcctcatcaagaacaccttcgagcagatcaatcccaacatcgaaatcacgtactggtcgtacgacggcgacacccaggataagaacgaagcggccgagcgccgcgacatgcgcgtgagcctgccggagctgctggcgaagggcttcaccgtgctgaactacaacagctactacctctacatcgtgccgaaggcgagcccgacgttctcgcaggacgccgccttcgccgccaaagacgtgatcaagaactgggatctgggcgtctgggatggccggaacaccaagaaccgcgtgcagaacacccatgagatcgccggggcggcgctgtcgatctggggcgaggatgcgaaggcgctcaaggacgagacgatccagaagaacaccaaaagcctgctcgaggccgtcatccacaagaccaacggcgacgagtga

SEQ ID NO: 16 - DNA, 69 bp, Staphylococcus aureus
  misc_feature: SaPSMa3 sequence added
atggagttcgtggcgaagctcttcaagttcttcaaggacctgctcgggaagttcctggggaataactga

SEQ ID NO: 17 - DNA, 135 bp, Staphylococcus aureus
  misc_feature: SaPAMb2 sequence added
atgaccggcctggccgaggcgatcgcgaataccgtccaggcggcccagcagcacgacagcgtcaagctgggcacctcgatcgtggacatcgtcgccaacggcgtgggcctgctgggcaaactcttcggcttctga

SEQ ID NO: 18 - DNA, 69 bp, Staphylococcus epidermidis
  misc_feature: SePSMa sequence added
atggcggacgtcatcgccaagatcgtcgagatcgtgaagggcctgatcgaccagttcacccagaagtga

SEQ ID NO: 19 - DNA, 228 bp, Levivirus MS2
  misc_feature: MS2 L sequence added
atggagacccggttcccgcagcagtcccagcaaaccccggccagcaccaaccgccgccgccccttcaagcacgaggactacccgtgccgccggcagcagcgcagctccaccctgtacgtgctgatcttcctggcgatcttcctgagcaagttcaccaaccagctgctgctgtccctgctggaggcggtcatccggaccgtcaccaccctgcagcagctgctgacctga

SEQ ID NO: 20 - DNA, 165 bp, Levivirus PRR1
  misc_feature: PRR1 L sequence added
atgtgcaaggtgtctactaaggtagactctaaactgactgagtcagttggacaactcaccataaggagctacctatggctacggaatatcctagcattagcaggacttcttttcgtaatccttcttgcgaccaatcatttatccatcgctatctacagtccgtaa

SEQ ID NO: 21 - DNA, 52 bp, Phikmvlikevirus LUZ19
  misc_feature: LUZ19 gp32 promoter (P32)
cgaccctgccctactccggccttaaacccacatccaaaagagagagaatcgc

SEQ ID NO: 22 - DNA, 96 bp, Phikmvlikevirus LUZ19
  misc_feature: LUZ19 gp32 terminator (T32)
tgccacgaaaccccgcacttcggtgtggggtttcttcaaagcctaacgacccgcgcagattccctgcgtgggtttttgcgctttaggagaaaccct

SEQ ID NO: 23 - DNA, 204 bp, Phikmvlikevirus LUZ19
  misc_feature: Wild type LUZ19 gp7 region
tacaaggtggtggcacccagctcggcggaaggtatcattgtgctggcgaccaagcagacgccggcgctagcccaagcagccgtcgtactgcacagcatgaaccctgcgcagtatcccgcaggttcggctatcctcaacacggcctggaagtgccgccgcctgggagtgggcgagtacgtcaagctcgtccaaggggaggaggac

SEQ ID NO: 24 - DNA, 321 bp, Phikmvlikevirus LUZ19
  misc_feature: Wild type LUZ19 gp18 region
gaatgccaaccgaagaagaacgcatgatccgctgtttactggcggatatccacgagccactggacctgctgttccccggcctccgtaccaaggcccatatggacccgcaagcagaggaactgtcgattcgaattgactacgaccatgcgaagctgggccgtatgggattctgccacgcggtatccctatatcaactgtccatatatggccgcgaggggatggtccgctacctgatgcaggagattccccgccgcgtgctggaaggtctgctggtcaaggcgcagcagtacagccaaagcaactggtacagcaaatgacgac

SEQ ID NO: 25 - DNA, 225 bp, Phikmvlikevirus LKD16
  misc_feature: Wild type LUZ19 gp49 and gp48-gp49 intergenic region
ggggacaccatgagcaaagccaaactacgagtcatcgccgacaccccggagctggagtcagtgctaaaagcattgctgaccgccacctacgctatcgaggacctgctcaacgaggccgtggctagcaaggtgctaaactcccgcctgggctggtccgcagtcggcgagtatgtcgaactgttcaaccgcacgcaatcccgcgtggccgggttgattcccgagtag

SEQ ID NO: 26 - DNA, 345 bp, Phikmvlikevirus LKD16
  misc_feature: Wild type LKD16 gp18 gene
gtgcgagtaccaactgaacacgagcgcaccctgcgctgcctgctccaagacatccacgggccgctgaatctgctgttcccaggtatccgggtgaaggtggaggaggcgtgcctcggatacttgggctacagggagcggggctattgggagctgcgcctccaggtggactacgaccacccgaagcttgggcacctccgctacagtcaggccgtgccggagtacgtgctgatcaacgaccgcgacagcatcatcaagtacctgatggaagcagtccctcggcaggtactagagggcatgctcaataaggcccaggaattcgtaaccaagaactggtattccctatga

SEQ ID NO: 27 - DNA, 4269 bp, Artificial Sequence
  Gene encoding NLS-FLAG-CAS9-His
atgcccaagaaaaagcggaaggtcggcgactacaaggatgacgatgacaagttggagcctggagagaagccctacaaatgccctgagtgcggaaagagcttcagccaatctggagccttgacccggcatcaacgaacgcatacacgagacaagaagtactccatcgggctggacatcgggacgaactccgtgggatgggccgtgatcacagacgaatacaaggtgccttccaagaagttcaaggtgctggggaacacggacagacactccatcaagaagaacctcatcggggccttgctcttcgactccggagaaaccgccgaagcaacgcgattgaaaagaaccgccagaagacgatacacacgacggaagaaccgcatctgctacctccaggagatcttcagcaacgagatggccaaggtggacgactcgttctttcatcgcctggaggagagcttcctggtggaggaagacaagaaacatgagcgccacccgatcttcgggaacatcgtggacgaagtggcctaccacgagaaataccccacgatctaccacttgcgcaagaaactcgtggactccacggacaaagcggacttgcggttgatctacttggccttggcccacatgatcaaatttcggggccacttcctgatcgagggcgacttgaatcccgacaattccgacgtggacaagctcttcatccagctggtgcagacctacaaccagctcttcgaggagaaccccatcaatgcctccggagtggacgccaaagccatcttgtccgcccgattgtccaaatccagacgcttggagaacttgatcgcacaacttcctggcgagaagaagaacggcctcttcggcaacttgatcgcgctgtcgctgggattgacgcctaacttcaagtccaacttcgacttggccgaggacgccaagttgcaactgtccaaggacacctacgacgacgacctcgacaacctgctggcccaaattggcgaccaatacgcggacttgtttttggcggccaagaacttgagcgacgccatcttgttgagcgacatcttgcgcgtgaatacggagatcaccaaagcccctttgtccgcctctatgatcaagcggtacgacgagcaccaccaagacttgaccctgttgaaagccctcgtgcggcaacaattgcccgagaagtacaaggagatcttcttcgaccagtccaagaacgggtacgccggctacatcgacggaggagcctcccaagaagagttctacaagttcatcaagcccatcctggagaagatggacggcaccgaggagttgctcgtgaagctgaaccgcgaagacttgttgcgaaaacagcggacgttcgacaatggcagcatcccccaccaaatccatttgggagagttgcacgccatcttgcgacggcaagaggacttctacccgttcctgaaggacaaccgcgagaaaatcgagaagatcctgacgttcagaatcccctactacgtgggacccttggcccgaggcaattcccggtttgcatggatgacgcgcaaaagcgaagagacgatcaccccctggaacttcgaagaagtggtcgacaaaggagcatccgcacagagcttcatcgagcgaatgacgaacttcgacaagaacctgcccaacgagaaggtgttgcccaagcattcgctgctgtacgagtacttcacggtgtacaacgagctgaccaaggtgaagtacgtgaccgagggcatgcgcaaacccgcgttcctgtcgggagagcaaaagaaggccattgtggacctgctgttcaagaccaaccggaaggtgaccgtgaaacagctgaaagaggactacttcaagaagatcgagtgcttcgactccgtggagatctccggcgtggaggaccgattcaatgcctccttgggaacctaccatgacctcctgaagatcatcaaggacaaggacttcctggacaacgaggagaacgaggacatcctggaggacatcgtgctgaccctgaccctgttcgaggaccgagagatgatcgaggaacggttgaaaacgtacgcccacttgttcgacgacaaggtgatgaagcagctgaaacgccgccgctacaccggatggggacgattgagccgcaaactgattaatggaattcgcgacaagcaatccggaaagaccatcctggacttcctgaagtccgacgggttcgccaaccgcaacttcatgcagctcatccacgacgactccttgaccttcaaggaggacatccagaaggcccaagtgtccggacaaggagactccttgcacgagcacatcgccaatttggccggatcccccgcaatcaaaaaaggcatcttgcaaaccgtgaaagtggtcgacgaactggtgaaggtgatgggacggcacaagcccgagaacatcgtgatcgaaatggcccgcgagaaccaaaccacccaaaaaggacagaagaactcccgagagcgcatgaagcggatcgaagagggcatcaaggagttgggctcccagatcctgaaggagcatcccgtggagaatacccaattgcaaaacgagaagctctacctctactacctccagaacgggcgggacatgtacgtcgaccaagagctggacatcaaccgcctctccgactacgatgtggatcatattgtgccccagagcttcctcaaggacgacagcatcgacaacaaggtcctgacgcgcagcgacaagaaccggggcaagtctgacaatgtgccttccgaagaagtcgtgaagaagatgaagaactactggcggcagctgctcaacgccaagctcatcacccaacggaagttcgacaacctgaccaaggccgagagaggaggattgtccgagttggacaaagccggcttcattaaacgccaactcgtggagacccgccagatcacgaagcacgtggcccaaatcttggactcccggatgaacacgaaatacgacgagaatgacaagctgatccgcgaggtgaaggtgatcacgctgaagtccaagctggtgagcgacttccggaaggacttccagttctacaaggtgcgggagatcaacaactaccatcacgcccatgacgcctacctgaacgccgtggtcggaaccgccctgatcaagaaataccccaagctggagtccgaattcgtgtacggagattacaaggtctacgacgtgcggaagatgatcgcgaagtccgagcaggagatcggcaaagccaccgccaagtacttcttttactccaacatcatgaacttcttcaagaccgagatcacgctcgccaacggcgagatccgcaagcgccccctgatcgagaccaacggcgagacgggagagattgtgtgggacaaaggaagagattttgccacagtgcgcaaggtgctgtccatgcctcaggtgaacatcgtgaagaagaccgaggtgcaaacaggagggttttccaaagagtccattttgcctaagaggaattccgacaagctcatcgcccgcaagaaggactgggaccccaagaagtacgggggcttcgactcccccacggtggcctactccgtgttggtggtggccaaagtggagaaagggaagagcaagaagctgaaatccgtgaaggagttgctcggaatcacgatcatggaacgatcgtcgttcgagaaaaaccccatcgacttcctcgaagccaaagggtacaaagaggtgaagaaggacctgatcatcaagctgcccaagtactccctgttcgagctggagaacggccgcaagcggatgctggcctccgccggggaactgcagaaagggaacgaattggccttgccctccaaatacgtgaacttcctctacttggcctcccattacgaaaagctcaaaggatcccctgaggacaatgagcagaagcaactcttcgtggaacaacacaagcactacctggacgagatcatcgagcagatcagcgagttctccaagcgcgtgatcctcgccgacgccaacctggacaaggtgctctccgcctacaacaagcaccgcgacaagcctatccgcgagcaagccgagaatatcattcacctgtttaccctgacgaatttgggagcccctgccgcctttaaatactttgacaccaccatcgaccgcaaaagatacacctccaccaaggaagtcttggacgccaccctcatccaccagtccatcacgggcctctacgagacgcgcatcgacctctcccaattgggcggcgaccatcatcaccaccaccactaa

SEQ ID NO: 28 - DNA, 507 bp, Inovirus M13MP18
  misc_feature: Wild type M13MP18 region replaced
atgaccatgattacgaattcgagctcggtacccggggatcctctagagtcgacctgcaggcatgcaagcttggcactggccgtcgttttacaacgtcgtgactgggaaaaccctggcgttacccaacttaatcgccttgcagcacatccccctttcgccagctggcgtaatagcgaagaggcccgcaccgatcgcccttcccaacagttgcgcagcctgaatggcgaatggcgctttgcctggtttccggcaccagaagcggtgccggaaagctggctggagtgcgatcttcctgaggccgatacggtcgtcgtcccctcaaactggcagatgcacggttacgatgcgcccatctacaccaacgtaacctatcccattacggtcaatccgccgtttgttcccacggagaatccgacgggttgttactcgctcacatttaatgttgatgaaagctggctacaggaaggccagacgcgaattatttttgatggcgttcctattggttaa

SEQ ID NO: 29 - DNA, 792 bp, Artificial Sequence
  Unknown
  misc_feature: Paprika sequence
  misc_feature: commercially available from DNA2.0
atggtgtcaaagggagaagaactgatcaaagagaatatgaggatgaaactctacatggaaggaactgtgaacaaccaccatttcaagtgcacgagcgagggtgaagggaaaccttacgaaggtacccagaccatgcggattaaggtcgtcgaaggaggaccactccccttcgcattcgacatcctggccacttccttcatgtacgggtcgcgcactttcatcaagtacccaaaagggatccccgacttcttcaagcagtcctttccggagggattcacttgggaacgcgtcactagatacgaggatggcggagtggtcaccgtgatgcaagacacctctttggaagatggatgcctggtgtaccacgtgcaagtcagaggagtgaactttccgagcaatgggccggtgatgcagaagaaaaccaagggctgggaaccgaacaccgaaatgctgtatccagcagacggaggcttggagggccggtccgacatggctctgaagcttgttggaggaggacatctgtcctgctcgttcgtgacgacctaccggagcaagaagccggcgaaaaaccttaagatgccggggatccacgcggtggatcatcgcctggaaaggctcgaggagtcagacaacgagatgtttgtcgtgcaacgcgagcacgccgtggcccgctactgtgatctcccttcaaagctgggccacaagctgaattccggcctccggtcgagagcccaggcttcgaattcagccgtggacggaactgcgggccctggttcgaccggaagccgatga

SEQ ID NO: 30 - DNA, 294 bp, lambdalike lambda
  misc_feature: Wild type E. coli phage
atggttcgtgcaaacaaacgcaacgaggctctacgaatcgagagtgcgttgcttaacaaaatcgcaatgcttggaactgagaagacagcggaagctgtgggcgttgataagtcgcagatcagcaggtggaagagggactggattccaaagttctcaatgctgcttgctgttcttgaatggggggtcgttgacgacgacatggctcgattggcgcgacaagttgctgcgattctcaccaataaaaaacgcccggcggcaaccgagcgttctgaacaaatccagatggagttctga

SEQ ID NO: 31 - protein, 1422 aa, Artificial Sequence
  Unknown
  misc_feature: NLS-FLAG-CAS9-His protein translated from SEQ ID NO:27
MPKKKRKVGDYKDDDDKLEPGEKPYKCPECGKSFSQSGALTRHQRTHTRDKKYSIGLDIGTNSVGWAVITDEYKVPSKKFKVLGNTDRHSIKKNLIGALLFDSGETAEATRLKRTARRRYTRRKNRICYLQEIFSNEMAKVDDSFFHRLEESFLVEEDKKHERHPIFGNIVDEVAYHEKYPTIYHLRKKLVDSTDKADLRLIYLALAHMIKFRGHFLIEGDLNPDNSDVDKLFIQLVQTYNQLFEENPINASGVDAKAILSARLSKSRRLENLIAQLPGEKKNGLFGNLIALSLGLTPNFKSNFDLAEDAKLQLSKDTYDDDLDNLLAQIGDQYADLFLAAKNLSDAILLSDILRVNTEITKAPLSASMIKRYDEHHQDLTLLKALVRQQLPEKYKEIFFDQSKNGYAGYIDGGASQEEFYKFIKPILEKMDGTEELLVKLNREDLLRKQRTFDNGSIPHQIHLGELHAILRRQEDFYPFLKDNREKIEKILTFRIPYYVGPLARGNSRFAWMTRKSEETITPWNFEEVVDKGASAQSFIERMTNFDKNLPNEKVLPKHSLLYEYFTVYNELTKVKYVTEGMRKPAFLSGEQKKAIVDLLFKTNRKVTVKQLKEDYFKKIECFDSVEISGVEDRFNASLGTYHDLLKIIKDKDFLDNEENEDILEDIVLTLTLFEDREMIEERLKTYAHLFDDKVMKQLKRRRYTGWGRLSRKLINGIRDKQSGKTILDFLKSDGFANRNFMQLIHDDSLTFKEDIQKAQVSGQGDSLHEHIANLAGSPAIKKGILQTVKVVDELVKVMGRHKPENIVIEMARENQTTQKGQKNSRERMKRIEEGIKELGSQILKEHPVENTQLQNEKLYLYYLQNGRDMYVDQELDINRLSDYDVDHIVPQSFLKDDSIDNKVLTRSDKNRGKSDNVPSEEVVKKMKNYWRQLLNAKLITQRKFDNLTKAERGGLSELDKAGFIKRQLVETRQITKHVAQILDSRMNTKYDENDKLIREVKVITLKSKLVSDFRKDFQFYKVREINNYHHAHDAYLNAVVGTALIKKYPKLESEFVYGDYKVYDVRKMIAKSEQEIGKATAKYFFYSNIMNFFKTEITLANGEIRKRPLIETNGETGEIVWDKGRDFATVRKVLSMPQVNIVKKTEVQTGGFSKESILPKRNSDKLIARKKDWDPKKYGGFDSPTVAYSVLVVAKVEKGKSKKLKSVKELLGITIMERSSFEKNPIDFLEAKGYKEVKKDLIIKLPKYSLFELENGRKRMLASAGELQKGNELALPSKYVNFLYLASHYEKLKGSPEDNEQKQLFVEQHKHYLDEIIEQISEFSKRVILADANLDKVLSAYNKHRDKPIREQAENIIHLFTLTNLGAPAAFKYFDTTIDRKRYTSTKEVLDATLIHQSITGLYETRIDLSQLGGDHHHHHH

SEQ ID NO: 32 - DNA, 909 bp, Cytomegalovirus HCMV
  misc_feature: HCMV RL13 fragment post-editing
atggactggcgatttacggttacgtggacgatactaatgtccgcgttgtcagaaagctgcaatcaaacctgttcttgtcaatgtccctgtagtactaccgttaactattcaactagtactgagacagccacatcaacatacagtacaacagttatcagcaataaaagcacttcagaatctataaattgctctactgcaactacaccagcaaacaccgtttctacaaaaccgtcggaaacaaccacacagatatccacaacgacgaacacaaacgttgagactaccacatgtaccaacaccaccacgaccgttacttgtgatggtttcaattatacagtccataaaagatgcgatcgcagttacgaggtaatcaacgtaacaggatacgttggtagcaacataactctaaaaaaatgcaatcagactgagaaatggcacaatgtagactggattcattatgagtaccccacgcataaaatgtgcgaattaggcaactatcaccaaaccacaccacggcacgacatatgttttgactgcaacgacacctccctaactatctacaacttaaccacaaaaaacgctggaaaatataccaggcgtcaccgtgataacggtcaagaagaaaattactacgtaacggtgttaattggagacacaacgttattcactcttggcacatgccctgtaagatataaagaatctacgaacactgaaaacaccattggaagtagcatcatagaaaccattgagaaagctaacattcccctgggaattcatgctgtatgggcaggcgtagtggtatcagtggcgcttatagcgttgtacatgggtagccatcgcattcccaaaaagccgcattacaccaaacttcccaaatatgatccagatgaattttggactaaggcttaa

SEQ ID NO: 33 - DNA, 630 bp, Cytomegalovirus HCMV
  misc_feature: HCMV RL13 fragment pre-editing
atggactggcgatttacggttacgtggaccgttacttgtgatggtttcaattatacagtccataaaagatgcgatcgcagttacgaggtaatcaacgtaacaggatacgttggtagcaacataactctaaaaaaatgcaatcagactgagaaatggcacaatgtagactggattcattatgagtaccccacgcataaaatgtgcgaattaggcaactatcaccaaaccacaccacggcacgacatatgttttgactgcaacgacacctccctaactatctacaacttaaccacaaaaaacgctggaaaatataccaggcgtcaccgtgataacggtcaagaagaaaattactacgtaacggtgttaattggagacacaacgttattcactcttggcacatgccctgtaagatataaagaatctacgaacactgaaaacaccattggaagtagcatcatagaaaccattgagaaagctaacattcccctgggaattcatgctgtatgggcaggcgtagtggtatcagtggcgcttatagcgttgtacatgggtagccatcgcattcccaaaaagccgcattacaccaaacttcccaaatatgatccagatgaattttggactaaggcttaa

SEQ ID NO: 34 - protein, 95 aa, Phikmvlikevirus LUZ19
  misc_feature: Wild type LUZ19 Gp13 protein sequence
MLALGAFDLSGLMVGSCLVVGGELKALCVDDRHSRQGIGAELVRAAELAGAEYLTCFEFLEPFYADLGWSTTHREANWTAGEPDVLHMRAPGHDV

SEQ ID NO: 35 - protein, 251 aa, Phikmvlikevirus LUZ19
  misc_feature: Wild type LUZ19 Gp38 protein sequence
MARFKNPETIHVADGVEAVFSLDFPFLRREDVFVQVDKILVTDYTWVDDTNIQLAVVPKKDQEVRIFRDTPAQVPDTQFSQDIPFLPRYIDANNKQLLYAVQEGINTANLALDGVLDAIRIAEEARRLAQEALDAANEALRRALGFAEIRTVTEDSDIDPSWRGYWNRCITADKPLTLTMQMEDPDAPWVEFSEVHFEQAGVRDLNIVAGPGVTINRLQNTTMQLYGENGVCTLKRLGANHWIVFGAMEDE

SEQ ID NO: 36 - protein, 301 aa, Phikmvlikevirus LUZ19
  misc_feature: Wild type LUZ19 Gp40 protein sequence
MFKTEVKGRYTLIRRKADGTPVETLEFDNIITNAGLDWIAAMDTDLMGEPVAVSTSTADPNPSAPAIPEVVQRTSASAPGGGTTSGLDGEWLFWRRRWRFPQGTLAGQVLATVGLICNSDRRFESNTGELIPKDTPLSYTRIKDAAGQPTTLVVAADEILDVQYEFRSRPVGTAEAKFVISGVERTFRLIPKPFANRANLSGERYIFYNTNPYINGKDASGGNVRDGQWQKKYPKYVRGSYKAQITLLAQVQNGNMAGGITGTEELQIYNGRNYVLDINPPVVKNNTQEFTVTLEFTVARA

SEQ ID NO: 37 - protein, 498 aa, Pseudomonas aeruginosa
  misc_feature: PyoS5 protein sequence
MSNDNEVPGSMVIVAQGPDDQYAYEVPPIDSAAVAGNMFGDLIQREIYLQKNIYYPVRSIFEQGTKEKKEINKKVSDQVDGLLKQITQGKREATRQERVDVMSAVLHKMESDLEGYKKTFTKGPFIDYEKQSSLSIYEAWVKIWEKNSWEERKKYPFQQLVRDELERAVAYYKQDSLSEAVKVLRQELNKQKALKEKEDLSQLERDYRTRKANLEMKVQSELDQAGSALPPLVSPTPEQWLERATRLVTQAIADKKQLQTTNNTLIKNSPTPLEKQKAIYNGELLVDEIASLQARLVKLNAETTRRRTEAERKAAEEQALQDAIKFTADFYKEVTEKFGARTSEMARQLAEGARGKNIRSSAEAIKSFEKHKDALNKKLSLKDRQAIAKAFDSLDKQMMAKSLEKFSKGFGVVGKAIDAASLYQEFKISTETGDWKPFFVKIETLAAGAAASWLVGIAFATATATPIGILGFALVMAVTGAMIDEDLLEKANNLVISI

SEQ ID NO: 38 - protein, 114 aa, Phikmvlikevirus LKD16
  misc_feature: LKD16 Gp18 protein sequence
MRVPTEHERTLRCLLQDIHGPLNLLFPGIRVKVEEACLGYLGYRERGYWELRLQVDYDHPKLGHLRYSQAVPEYVLINDRDSIIKYLMEAVPRQVLEGMLNKAQEFVTKNWYSL

SEQ ID NO: 39 - protein, 769 aa, Phikmvlikevirus LKA1
  misc_feature: LKA1 Gp49 protein sequence
MAQTPSTWADYVGDGVEDTFQVTFPYQKQQEVFVTVGGDPAAFTFISAGWIQLAAVPVNGAAIRVRRSTEAFEPRHEFANGVPLLPRFIDENNTQFLYTVQEAVNETHGIASEALSVAEEARGIAQAASDKVDAATIDSAHQLRLDLADPAKGPGLLGYDRDVSYPVGSVGQSLQFLEMGRVTPAQFGAVGDGASHPLSERYATLAEAQTVYPHAVALSDEIDWAALQAAVDSGAPVHIPSGDYQINRGISSTGSLQIAGDGATSIIRPTAAFTGTSVLSCVGSLVALPNISSVSAGSLTIDFASTPNLVAGDVFIIYNPTDSSFSGFRTSYRAGEFCEVRAVSGNTVTIRSALYAAYDGATVAIYKVVSGVVDIASIQIVGGTVPMNGLLVEAVVSPRVDDVTVTLANNAGVYFARCYDAKITNSNISNIGDGGDDYGIIFGNCHDGGADNCKVYARRHAIATGGDAEVGCVPVRNVRMRNCTLRNDITSGTHCADFHGNAEDCSYENCTIYGGATWQGKDISYRHCTITNASGGWIVISAEILGGTFLLDQCTLYTTGDPQPGNRGVIDVGGNSAVLTTNTTQPCNFLIQGGSLRAPSLSTSSYLLRARLEGSTVPVNIQYSGQAIDVGSLGKVLQLDITSGSTSPEYLIVENLAGLPSGITLASAAGGFASAPMRMPVLGGRVQVTTATNASSVTAPVTFRYIYPKAPTVQVTKTDRSYAGNRVGVAIANPTSASGATLGLFTDDGTNFSSAVTNQLNWQAGIYEV

SEQ ID NO: 40 - protein, 651 aa, Phikmvlikevirus NTUH-K2044-K1-1
  misc_feature: NTUH-K2044-K1-1 Gp34 protein sequence
MALIRLVAPERVFSDLASMVAYPNFQVQDKITLLGSAGGDFTFTTTASVVDNGTVFAVPGGYLLRKFVGPAYSSWFSNWTGIVTFMSAPNRHLVVDTVLQATSVLNIKSNSTLEFTDTGRILPDAAVARQVLNITGSAPSVFVPLAADAAAGSKVITVAAGALSAVKGTYLYLRSNKLCDGGPNTYGVKISQIRKVVGVSTSGGVTSIRLDKALHYNYYLSDAAEVGIPTMVENVTLVSPYINEFGYDDLNRFFTSGISANFAADLHIQDGVIIGNKRPGASDIEGRSAIKFNNCVDSTVKGTCFYNIGWYGVEVLGCSEDTEVHDIHAMDVRHAISLNWQSTADGDKWGEPIEFLGVNCEAYSTTQAGFDTHDIGKRVKFVRCVSYDSADDGFQARTNGVEYLNCRAYRAAMDGFASNTGVAFPIYRECLAYDNVRSGFNCSYGGGYVYDCEAHGSQNGVRINGGRVKGGRYTRNSSSHIFVTKDVAETAQTSLEIDGVSMRYDGTGRAVYFHGTVGIDPTLVSMSNNDMTGHGLFWALLSGYTVQPTPPRMSRNLLDDTGIRGVATLVAGEATVNARVRGNFGSVANSFKWVSEVKLTRLTFPSSAGALTVTSVAQNQDVPTPNPDLNSFVIRSSNAADVSQVAWEVYL

SEQ ID NO: 41 - protein, 727 aa, T7-like Pp15
  misc_feature: Pp15 Gp44 protein sequence
MARTIVQNALTGGQQDFEVPFDYILQRFVKLTLIGDGNRQELVLGTDFRFIGPRTVRTNVFWGPAQGYTSIEIRRVTSASDRRVEFSDGSILTAGDLNIAQLQAIHIAEEARDSATENLSPDADGNYDARGARIYNLGDAVQPKDAVNRYTLDLAIAAALAMNTGNPNNAQNISYTPNGPGQSIRSVEGRLRDAVFVSDYMTTPRDGVTSNQQDLEKALAAANAKGADLFWPDDIPFFSTSPLALIHAVYHVGRGVINANGTLFYVNPKNGQHNRLHVSPGGTGDGLAAGRPLGTIWSALAALNMRAPLTTRWSLEMTAGAYNEAVTLPNYLTSCNDYLAFNWPNTGQERMEPTAYPSALDGTGQTGLTGFHTGIGNRITINNVCMSNWYDTALTPTQQVRRAFVVGAYSTAYVVNCAFIYNGIASVSVLPGGTAIVTGGIVDGGRFGLDNTGGRLSLTATKSNYTQVRNCLEYGLYSKHDASTVMDNTEFRNCGNHPAAVAYGAAIFAYKFNCSVDTRGVKFYGNNIAQHCRGGITSDNPGDPDIYGTGADANKRLFLCTGGGSDDIQFYEARRVMDITKRTGGGSTTASVSSLLLAAVASVRKGYFAHNDQVIRMTLMFRATGSAGIFTPTLRTPLGTIPLGSFRVASGQYGEIKLTIRPTLTSDGLIVGFSCINAVQNLGSSVGQIIVSGTVDLRTVDQLVEMWGYSEAGGTASYIQGLIELVG

SEQ ID NO: 42 - protein, 362 aa, Aggregatibacter actinomycetemcomitans
  misc_feature: DspB protein sequence
MNCCVKGNSIYPQKTSTKQTGLMLDIARHFYSPEVIKSFIDTISLSGGNFLHLHFSDHENYAIESHLLNQRAENAVQGKDGIYINPYTGKPFLSYRQLDDIKAYAKAKGIELIPELDSPNHMTAIFKLVQKDRGVKYLQGLKSRQVDDEIDITNADSITFMQSLMSEVIDIFGDTSQHFHIGGDEFGYSVESNHEFITYANKLSYFLEKKGLKTRMWNDGLIKNTFEQINPNIEITYWSYDGDTQDKNEAAERRDMRVSLPELLAKGFTVLNYNSYYLYIVPKASPTFSQDAAFAAKDVIKNWDLGVWDGRNTKNRVQNTHEIAGAALSIWGEDAKALKDETIQKNTKSLLEAVIHKTNGDE

SEQ ID NO: 43 - protein, 22 aa, Staphylococcus aureus
  misc_feature: SaPSMa3 protein sequence
MEFVAKLFKFFKDLLGKFLGNN

SEQ ID NO: 44 - protein, 44 aa, Staphylococcus aureus
  misc_feature: SaPAMb2 protein sequence
MTGLAEAIANTVQAAQQHDSVKLGTSIVDIVANGVGLLGKLFGF

SEQ ID NO: 45 - protein, 22 aa, Staphylococcus epidermidis
  misc_feature: SePSMa protein sequence
MADVIAKIVEIVKGLIDQFTQK

SEQ ID NO: 46 - protein, 75 aa, Levivirus MS2
  misc_feature: MS2 L protein sequence
METRFPQQSQQTPASTNRRRPFKHEDYPCRRQQRSSTLYVLIFLAIFLSKFTNQLLLSLLEAVIRTVTTLQQLLT

SEQ ID NO: 47 - protein, 54 aa, Levivirus PRR1
  misc_feature: PRR1 L protein sequence
MCKVSTKVDSKLTESVGQLTIRSYLWLRNILALAGLLFVILLATNHLSIAIYSP

SEQ ID NO: 48 - protein, 106 aa, Phikmvlikevirus LUZ19
  misc_feature: LUZ19 Gp18 protein sequence
MRMPTEEERMIRCLLADIHEPLDLLFPGLRTKAHMDPQAEELSIRIDYDHAKLGRMGFCHAVSLYQLSIYGREGMVRYLMQEIPRRVLEGLLVKAQQYSQSNWYSK

SEQ ID NO: 49 - protein, 71 aa, Phikmvlikevirus LUZ19
  misc_feature: LUZ19 Gp49 protein sequence
MSKAKLRVIADTPELESVLKALLTATYAIEDLLNEAVASKVLNSRLGWSAVGEYVELFNRTQSRVAGLIPE

SEQ ID NO: 50 - DNA, 321 bp, Phikmvlikevirus LUZ19
  misc_feature: LUZ19 gp18 gene sequence
atgagaatgccaaccgaagaagaacgcatgatccgctgtttactggcggatatccacgagccactggacctgctgttccccggcctccgtaccaaggcccatatggacccgcaagcagaggaactgtcgattcgaattgactacgaccatgcgaagctgggccgtatgggattctgccacgcggtatccctatatcaactgtccatatatggccgcgaggggatggtccgctacctgatgcaggagattccccgccgcgtgctggaaggtctgctggtcaaggcgcagcagtacagccaaagcaactggtacagcaaatga

SEQ ID NO: 51 - DNA, 216 bp, Phikmvlikevirus LUZ19
  misc_feature: LUZ19 Gp49 protein sequence
atgagcaaagccaaactacgagtcatcgccgacaccccggagctggagtcagtgctaaaagcattgctgaccgccacctacgctatcgaggacctgctcaacgaggccgtggctagcaaggtgctaaactcccgcctgggctggtccgcagtcggcgagtatgtcgaactgttcaaccgcacgcaatcccgcgtggccgggttgattcccgagtag